European Patent Application EP 4 560 021 A1, published May 28, 2025. Title: MRNA FOR SARS-COV-2 S PROTEIN AND USE THEREOF. Applicant: Shenzhen Shenxin Biotechnology Co., Ltd. Application CN. The sequence listing filed with the application follows.

SEQUENCE LISTING (76 sequences)

SEQ ID NO: 1 - DNA, 7040 bp, synthetic construct
  misc_feature 1..7040
  source 1..7040: mol_type = other DNA
gacggatcgggagatctcccgatcccctatggtgcactctcagtacaatctgctctgatgccgcatagttaagccagtatctgctccctgcttgtgtgttggaggtcgctgagtagtgcgcgagcaaaatttaagctacaacaaggcaaggcttgaccgacaattgcatgaagaatctgcttagggttaggcgttttgcgctgcttcgcgatgtacgggccagatatacgcgttgacattgattattgactagttattaatagtaatcaattacggggtcattagttcatagcccatatatggagttccgcgttacataacttacggtaaatggcccgcctggctgaccgcccaacgacccccgcccattgacgtcaataatgacgtatgttcccatagtaacgccaatagggactttccattgacgtcaatgggtggagtatttacggtaaactgcccacttggcagtacatcaagtgtatcatatgccaagtacgccccctattgacgtcaatgacggtaaatggcccgcctggcattatgcccagtacatgaccttatgggactttcctacttggcagtacatctacgtattagtcatcgctattaccatggtgatgcggttttggcagtacatcaatgggcgtggatagcggtttgactcacggggatttccaagtctccaccccattgacgtcaatgggagtttgttttggcaccaaaatcaacgggactttccaaaatgtcgtaacaactccgccccattgacgcaaatgggcggtaggcgtgtacggtgggaggtctatataagcagagctctctggctaactagagaacccactgcttactggcttatcgaaattaatacgactcactatagggagacccaagcttggcattccggtactgttggtaaagccaccatggaagacgccaaaaacataaagaaaggcccggcgccattctatccgctggaagatggaaccgctggagagcaactgcataaggctatgaagagatacgccctggttcctggaacaattgcttttacagatgcacatatcgaggtggacatcacttacgctgagtacttcgaaatgtccgttcggttggcagaagctatgaaacgatatgggctgaatacaaatcacagaatcgtcgtatgcagtgaaaactctcttcaattctttatgccggtgttgggcgcgttatttatcggagttgcagttgcgcccgcgaacgacatttataatgaacgtgaattgctcaacagtatgggcatttcgcagcctaccgtggtgttcgtttccaaaaaggggttgcaaaaaattttgaacgtgcaaaaaaagctcccaatcatccaaaaaattattatcatggattctaaaacggattaccagggatttcagtcgatgtacacgttcgtcacatctcatctacctcccggttttaatgaatacgattttgtgccagagtccttcgatagggacaagacaattgcactgatcatgaactcctctggatctactggtctgcctaaaggtgtcgctctgcctcatagaactgcctgcgtgagattctcgcatgccagagatcctatttttggcaatcaaatcattccggatactgcgattttaagtgttgttccattccatcacggttttggaatgtttactacactcggatatttgatatgtggatttcgagtcgtcttaatgtatagatttgaagaagagctgtttctgaggagccttcaggattacaagattcaaagtgcgctgctggtgccaaccctattctccttcttcgccaaaagcactctgattgacaaatacgatttatctaatttacacgaaattgcttctggtggcgctcccctctctaaggaagtcggggaagcggttgccaagaggttccatctgccaggtatcaggcaaggatatgggctcactgagactacatcagctattctgattacacccgagggggatgataaaccgggcgcggtcggtaaagttgttccattttttgaagcgaaggttgtggatctggataccgggaaaacgctgggcgttaatcaaagaggcgaactgtgtgtgagaggtcctatgattatgtccggttatgtaaacaatccggaagcgaccaacgccttgattgacaaggatggatggctacattctggagacatagcttactgggacgaagacgaacacttcttcatcgttgaccgcctgaagtctctgattaagtacaaaggctatcaggtggctcccgctgaattggaatccatcttgctccaacaccccaacatcttcgacgcaggtgtcgcaggtcttcccgacgatgacgccggtgaacttcccgccgccgttgttgttttggagcacggaaagacgatgacggaaaaagagatcgtggattacgtcgccagtcaagtaacaaccgcgaaaaagttgcgcggaggagttgtgtttgtggacgaagtaccgaaaggtcttaccggaaaactcgacgcaagaaaaatcagagagatcctcataaaggccaagaagggcggaaagatcgccgtgtaattctagagggccctattctatagtgtcacctaaatgctagagctcgctgatcagcctcgactgtgccttctagttgccagccatctgttgtttgcccctcccccgtgccttccttgaccctggaaggtgccactcccactgtcctttcctaataaaatgaggaaattgcatcgcattgtctgagtaggtgtcattctattctggggggtggggtggggcaggacagcaagggggaggattgggaagacaatagcaggcatgctggggatgcggtgggctctatggcttctgaggcggaaagaaccagctggggctctagggggtatccccacgcgccctgtagcggcgcattaagcgcggcgggtgtggtggttacgcgcagcgtgaccgctacacttgccagcgccctagcgcccgctcctttcgctttcttcccttcctttctcgccacgttcgccggctttccccgtcaagctctaaatcgggggctccctttagggttccgatttagtgctttacggcacctcgaccccaaaaaacttgattagggtgatggttcacgtagtgggccatcgccctgatagacggtttttcgccctttgacgttggagtccacgttctttaatagtggactcttgttccaaactggaacaacactcaaccctatctcggtctattcttttgatttataagggattttgccgatttcggcctattggttaaaaaatgagctgatttaacaaaaatttaacgcgaattaattctgtggaatgtgtgtcagttagggtgtggaaagtccccaggctccccagcaggcagaagtatgcaaagcatgcatctcaattagtcagcaaccaggtgtggaaagtccccaggctccccagcaggcagaagtatgcaaagcatgcatctcaattagtcagcaaccatagtcccgcccctaactccgcccatcccgcccctaactccgcccagttccgcccattctccgccccatggctgactaattttttttatttatgcagaggccgaggccgcctctgcctctgagctattccagaagtagtgaggaggcttttttggaggcctaggcttttgcaaaaagctcccgggagcttgtatatccattttcggatctgatcaagagacaggatgaggatcgtttcgcatgattgaacaagatggattgcacgcaggttctccggccgcttgggtggagaggctattcggctatgactgggcacaacagacaatcggctgctctgatgccgccgtgttccggctgtcagcgcaggggcgcccggttctttttgtcaagaccgacctgtccggtgccctgaatgaactgcaggacgaggcagcgcggctatcgtggctggccacgacgggcgttccttgcgcagctgtgctcgacgttgtcactgaagcgggaagggactggctgctattgggcgaagtgccggggcaggatctcctgtcatctcaccttgctcctgccgagaaagtatccatcatggctgatgcaatgcggcggctgcatacgcttgatccggctacctgcccattcgaccaccaagcgaaacatcgcatcgagcgagcacgtactcggatggaagccggtcttgtcgatcaggatgatctggacgaagagcatcaggggctcgcgccagccgaactgttcgccaggctcaaggcgcgcatgcccgacggcgaggatctcgtcgtgacccatggcgatgcctgcttgccgaatatcatggtggaaaatggccgcttttctggattcatcgactgtggccggctgggtgtggcggaccgctatcaggacatagcgttggctacccgtgatattgctgaagagcttggcggcgaatgggctgaccgcttcctcgtgctttacggtatcgccgctcccgattcgcagcgcatcgccttctatcgccttcttgacgagttcttctgagcgggactctggggttcgaaatgaccgaccaagcgacgcccaacctgccatcacgagatttcgattccaccgccgccttctatgaaaggttgggcttcggaatcgttttccgggacgccggctggatgatcctccagcgcggggatctcatgctggagttcttcgcccaccccaacttgtttattgcagcttataatggttacaaataaagcaatagcatcacaaatttcacaaataaagcatttttttcactgcattctagttgtggtttgtccaaactcatcaatgtatcttatcatgtctgtataccgtcgacctctagctagagcttggcgtaatcatggtcatagctgtttcctgtgtgaaattgttatccgctcacaattccacacaacatacgagccggaagcataaagtgtaaagcctggggtgcctaatgagtgagctaactcacattaattgcgttgcgctcactgcccgctttccagtcgggaaacctgtcgtgccagctgcattaatgaatcggccaacgcgcggggagaggcggtttgcgtattgggcgctcttccgcttcctcgctcactgactcgctgcgctcggtcgttcggctgcggcgagcggtatcagctcactcaaaggcggtaatacggttatccacagaatcaggggataacgcaggaaagaacatgtgagcaaaaggccagcaaaaggccaggaaccgtaaaaaggccgcgttgctggcgtttttccataggctccgcccccctgacgagcatcacaaaaatcgacgctcaagtcagaggtggcgaaacccgacaggactataaagataccaggcgtttccccctggaagctccctcgtgcgctctcctgttccgaccctgccgcttaccggatacctgtccgcctttctcccttcgggaagcgtggcgctttctcatagctcacgctgtaggtatctcagttcggtgtaggtcgttcgctccaagctgggctgtgtgcacgaaccccccgttcagcccgaccgctgcgccttatccggtaactatcgtcttgagtccaacccggtaagacacgacttatcgccactggcagcagccactggtaacaggattagcagagcgaggtatgtaggcggtgctacagagttcttgaagtggtggcctaactacggctacactagaagaacagtatttggtatctgcgctctgctgaagccagttaccttcggaaaaagagttggtagctcttgatccggcaaacaaaccaccgctggtagcggtggtttttttgtttgcaagcagcagattacgcgcagaaaaaaaggatctcaagaagatcctttgatcttttctacggggtctgacgctcagtggaacgaaaactcacgttaagggattttggtcatgagattatcaaaaaggatcttcacctagatccttttaaattaaaaatgaagttttaaatcaatctaaagtatatatgagtaaacttggtctgacagttaccaatgcttaatcagtgaggcacctatctcagcgatctgtctatttcgttcatccatagttgcctgactccccgtcgtgtagataactacgatacgggagggcttaccatctggccccagtgctgcaatgataccgcgagacccacgctcaccggctccagatttatcagcaataaaccagccagccggaagggccgagcgcagaagtggtcctgcaactttatccgcctccatccagtctattaattgttgccgggaagctagagtaagtagttcgccagttaatagtttgcgcaacgttgttgccattgctacaggcatcgtggtgtcacgctcgtcgtttggtatggcttcattcagctccggttcccaacgatcaaggcgagttacatgatcccccatgttgtgcaaaaaagcggttagctccttcggtcctccgatcgttgtcagaagtaagttggccgcagtgttatcactcatggttatggcagcactgcataattctcttactgtcatgccatccgtaagatgcttttctgtgactggtgagtactcaaccaagtcattctgagaatagtgtatgcggcgaccgagttgctcttgcccggcgtcaatacgggataataccgcgccacatagcagaactttaaaagtgctcatcattggaaaacgttcttcggggcgaaaactctcaaggatcttaccgctgttgagatccagttcgatgtaacccactcgtgcacccaactgatcttcagcatcttttactttcaccagcgtttctgggtgagcaaaaacaggaaggcaaaatgccgcaaaaaagggaataagggcgacacggaaatgttgaatactcatactcttcctttttcaatattattgaagcatttatcagggttattgtctcatgagcggatacatatttgaatgtatttagaaaaataaacaaataggggttccgcgcacatttccccgaaaagtgccacctgacgtc

SEQ ID NO: 2 - DNA, 7041 bp, synthetic construct
  misc_feature 1..7041: note = plasmid
  source 1..7041: mol_type = other DNA
gacggatcgggagatctcccgatcccctatggtgcactctcagtacaatctgctctgatgccgcatagttaagccagtatctgctccctgcttgtgtgttggaggtcgctgagtagtgcgcgagcaaaatttaagctacaacaaggcaaggcttgaccgacaattgcatgaagaatctgcttagggttaggcgttttgcgctgcttcgcgatgtacgggccagatatacgcgttgacattgattattgactagttattaatagtaatcaattacggggtcattagttcatagcccatatatggagttccgcgttacataacttacggtaaatggcccgcctggctgaccgcccaacgacccccgcccattgacgtcaataatgacgtatgttcccatagtaacgccaatagggactttccattgacgtcaatgggtggagtatttacggtaaactgcccacttggcagtacatcaagtgtatcatatgccaagtacgccccctattgacgtcaatgacggtaaatggcccgcctggcattatgcccagtacatgaccttatgggactttcctacttggcagtacatctacgtattagtcatcgctattaccatggtgatgcggttttggcagtacatcaatgggcgtggatagcggtttgactcacggggatttccaagtctccaccccattgacgtcaatgggagtttgttttggcaccaaaatcaacgggactttccaaaatgtcgtaacaactccgccccattgacgcaaatgggcggtaggcgtgtacggtgggaggtctatataagcagagctctctggctaactagagaacccactgcttactggcttatcgaaattaatacgactcactatagggaaagcttgatcagaacggatccgccaccatggaagacgccaaaaacataaagaaaggcccggcgccattctatccgctggaagatggaaccgctggagagcaactgcataaggctatgaagagatacgccctggttcctggaacaattgcttttacagatgcacatatcgaggtggacatcacttacgctgagtacttcgaaatgtccgttcggttggcagaagctatgaaacgatatgggctgaatacaaatcacagaatcgtcgtatgcagtgaaaactctcttcaattctttatgccggtgttgggcgcgttatttatcggagttgcagttgcgcccgcgaacgacatttataatgaacgtgaattgctcaacagtatgggcatttcgcagcctaccgtggtgttcgtttccaaaaaggggttgcaaaaaattttgaacgtgcaaaaaaagctcccaatcatccaaaaaattattatcatggattctaaaacggattaccagggatttcagtcgatgtacacgttcgtcacatctcatctacctcccggttttaatgaatacgattttgtgccagagtccttcgatagggacaagacaattgcactgatcatgaactcctctggatctactggtctgcctaaaggtgtcgctctgcctcatagaactgcctgcgtgagattctcgcatgccagagatcctatttttggcaatcaaatcattccggatactgcgattttaagtgttgttccattccatcacggttttggaatgtttactacactcggatatttgatatgtggatttcgagtcgtcttaatgtatagatttgaagaagagctgtttctgaggagccttcaggattacaagattcaaagtgcgctgctggtgccaaccctattctccttcttcgccaaaagcactctgattgacaaatacgatttatctaatttacacgaaattgcttctggtggcgctcccctctctaaggaagtcggggaagcggttgccaagaggttccatctgccaggtatcaggcaaggatatgggctcactgagactacatcagctattctgattacacccgagggggatgataaaccgggcgcggtcggtaaagttgttccattttttgaagcgaaggttgtggatctggataccgggaaaacgctgggcgttaatcaaagaggcgaactgtgtgtgagaggtcctatgattatgtccggttatgtaaacaatccggaagcgaccaacgccttgattgacaaggatggatggctacattctggagacatagcttactgggacgaagacgaacacttcttcatcgttgaccgcctgaagtctctgattaagtacaaaggctatcaggtggctcccgctgaattggaatccatcttgctccaacaccccaacatcttcgacgcaggtgtcgcaggtcttcccgacgatgacgccggtgaacttcccgccgccgttgttgttttggagcacggaaagacgatgacggaaaaagagatcgtggattacgtcgccagtcaagtaacaaccgcgaaaaagttgcgcggaggagttgtgtttgtggacgaagtaccgaaaggtcttaccggaaaactcgacgcaagaaaaatcagagagatcctcataaaggccaagaagggcggaaagatcgccgtgtaaggtacccgatcagattctagagggccctattctatagtgtcacctaaatgctagagctcgctgatcagcctcgactgtgccttctagttgccagccatctgttgtttgcccctcccccgtgccttccttgaccctggaaggtgccactcccactgtcctttcctaataaaatgaggaaattgcatcgcattgtctgagtaggtgtcattctattctggggggtggggtggggcaggacagcaagggggaggattgggaagacaatagcaggcatgctggggatgcggtgggctctatggcttctgaggcggaaagaaccagctggggctctagggggtatccccacgcgccctgtagcggcgcattaagcgcggcgggtgtggtggttacgcgcagcgtgaccgctacacttgccagcgccctagcgcccgctcctttcgctttcttcccttcctttctcgccacgttcgccggctttccccgtcaagctctaaatcgggggctccctttagggttccgatttagtgctttacggcacctcgaccccaaaaaacttgattagggtgatggttcacgtagtgggccatcgccctgatagacggtttttcgccctttgacgttggagtccacgttctttaatagtggactcttgttccaaactggaacaacactcaaccctatctcggtctattcttttgatttataagggattttgccgatttcggcctattggttaaaaaatgagctgatttaacaaaaatttaacgcgaattaattctgtggaatgtgtgtcagttagggtgtggaaagtccccaggctccccagcaggcagaagtatgcaaagcatgcatctcaattagtcagcaaccaggtgtggaaagtccccaggctccccagcaggcagaagtatgcaaagcatgcatctcaattagtcagcaaccatagtcccgcccctaactccgcccatcccgcccctaactccgcccagttccgcccattctccgccccatggctgactaattttttttatttatgcagaggccgaggccgcctctgcctctgagctattccagaagtagtgaggaggcttttttggaggcctaggcttttgcaaaaagctcccgggagcttgtatatccattttcggatctgatcaagagacaggatgaggatcgtttcgcatgattgaacaagatggattgcacgcaggttctccggccgcttgggtggagaggctattcggctatgactgggcacaacagacaatcggctgctctgatgccgccgtgttccggctgtcagcgcaggggcgcccggttctttttgtcaagaccgacctgtccggtgccctgaatgaactgcaggacgaggcagcgcggctatcgtggctggccacgacgggcgttccttgcgcagctgtgctcgacgttgtcactgaagcgggaagggactggctgctattgggcgaagtgccggggcaggatctcctgtcatctcaccttgctcctgccgagaaagtatccatcatggctgatgcaatgcggcggctgcatacgcttgatccggctacctgcccattcgaccaccaagcgaaacatcgcatcgagcgagcacgtactcggatggaagccggtcttgtcgatcaggatgatctggacgaagagcatcaggggctcgcgccagccgaactgttcgccaggctcaaggcgcgcatgcccgacggcgaggatctcgtcgtgacccatggcgatgcctgcttgccgaatatcatggtggaaaatggccgcttttctggattcatcgactgtggccggctgggtgtggcggaccgctatcaggacatagcgttggctacccgtgatattgctgaagagcttggcggcgaatgggctgaccgcttcctcgtgctttacggtatcgccgctcccgattcgcagcgcatcgccttctatcgccttcttgacgagttcttctgagcgggactctggggttcgaaatgaccgaccaagcgacgcccaacctgccatcacgagatttcgattccaccgccgccttctatgaaaggttgggcttcggaatcgttttccgggacgccggctggatgatcctccagcgcggggatctcatgctggagttcttcgcccaccccaacttgtttattgcagcttataatggttacaaataaagcaatagcatcacaaatttcacaaataaagcatttttttcactgcattctagttgtggtttgtccaaactcatcaatgtatcttatcatgtctgtataccgtcgacctctagctagagcttggcgtaatcatggtcatagctgtttcctgtgtgaaattgttatccgctcacaattccacacaacatacgagccggaagcataaagtgtaaagcctggggtgcctaatgagtgagctaactcacattaattgcgttgcgctcactgcccgctttccagtcgggaaacctgtcgtgccagctgcattaatgaatcggccaacgcgcggggagaggcggtttgcgtattgggcgctcttccgcttcctcgctcactgactcgctgcgctcggtcgttcggctgcggcgagcggtatcagctcactcaaaggcggtaatacggttatccacagaatcaggggataacgcaggaaagaacatgtgagcaaaaggccagcaaaaggccaggaaccgtaaaaaggccgcgttgctggcgtttttccataggctccgcccccctgacgagcatcacaaaaatcgacgctcaagtcagaggtggcgaaacccgacaggactataaagataccaggcgtttccccctggaagctccctcgtgcgctctcctgttccgaccctgccgcttaccggatacctgtccgcctttctcccttcgggaagcgtggcgctttctcatagctcacgctgtaggtatctcagttcggtgtaggtcgttcgctccaagctgggctgtgtgcacgaaccccccgttcagcccgaccgctgcgccttatccggtaactatcgtcttgagtccaacccggtaagacacgacttatcgccactggcagcagccactggtaacaggattagcagagcgaggtatgtaggcggtgctacagagttcttgaagtggtggcctaactacggctacactagaagaacagtatttggtatctgcgctctgctgaagccagttaccttcggaaaaagagttggtagctcttgatccggcaaacaaaccaccgctggtagcggtggtttttttgtttgcaagcagcagattacgcgcagaaaaaaaggatctcaagaagatcctttgatcttttctacggggtctgacgctcagtggaacgaaaactcacgttaagggattttggtcatgagattatcaaaaaggatcttcacctagatccttttaaattaaaaatgaagttttaaatcaatctaaagtatatatgagtaaacttggtctgacagttaccaatgcttaatcagtgaggcacctatctcagcgatctgtctatttcgttcatccatagttgcctgactccccgtcgtgtagataactacgatacgggagggcttaccatctggccccagtgctgcaatgataccgcgagacccacgctcaccggctccagatttatcagcaataaaccagccagccggaagggccgagcgcagaagtggtcctgcaactttatccgcctccatccagtctattaattgttgccgggaagctagagtaagtagttcgccagttaatagtttgcgcaacgttgttgccattgctacaggcatcgtggtgtcacgctcgtcgtttggtatggcttcattcagctccggttcccaacgatcaaggcgagttacatgatcccccatgttgtgcaaaaaagcggttagctccttcggtcctccgatcgttgtcagaagtaagttggccgcagtgttatcactcatggttatggcagcactgcataattctcttactgtcatgccatccgtaagatgcttttctgtgactggtgagtactcaaccaagtcattctgagaatagtgtatgcggcgaccgagttgctcttgcccggcgtcaatacgggataataccgcgccacatagcagaactttaaaagtgctcatcattggaaaacgttcttcggggcgaaaactctcaaggatcttaccgctgttgagatccagttcgatgtaacccactcgtgcacccaactgatcttcagcatcttttactttcaccagcgtttctgggtgagcaaaaacaggaaggcaaaatgccgcaaaaaagggaataagggcgacacggaaatgttgaatactcatactcttcctttttcaatattattgaagcatttatcagggttattgtctcatgagcggatacatatttgaatgtatttagaaaaataaacaaataggggttccgcgcacatttccccgaaaagtgccacctgacgtc

SEQ ID NO: 3 - DNA, 7202 bp, synthetic construct
  misc_feature 1..7202: note = plasmid
  source 1..7202: mol_type = other DNA
gacggatcgggagatctcccgatcccctatggtgcactctcagtacaatctgctctgatgccgcatagttaagccagtatctgctccctgcttgtgtgttggaggtcgctgagtagtgcgcgagcaaaatttaagctacaacaaggcaaggcttgaccgacaattgcatgaagaatctgcttagggttaggcgttttgcgctgcttcgcgatgtacgggccagatatacgcgttgacattgattattgactagttattaatagtaatcaattacggggtcattagttcatagcccatatatggagttccgcgttacataacttacggtaaatggcccgcctggctgaccgcccaacgacccccgcccattgacgtcaataatgacgtatgttcccatagtaacgccaatagggactttccattgacgtcaatgggtggagtatttacggtaaactgcccacttggcagtacatcaagtgtatcatatgccaagtacgccccctattgacgtcaatgacggtaaatggcccgcctggcattatgcccagtacatgaccttatgggactttcctacttggcagtacatctacgtattagtcatcgctattaccatggtgatgcggttttggcagtacatcaatgggcgtggatagcggtttgactcacggggatttccaagtctccaccccattgacgtcaatgggagtttgttttggcaccaaaatcaacgggactttccaaaatgtcgtaacaactccgccccattgacgcaaatgggcggtaggcgtgtacggtgggaggtctatataagcagagctctctggctaactagagaacccactgcttactggcttatcgaaattaatacgactcactatagggaaagctttaatacgactcactataggacagatcgcctggagacgccatccacgctgttttgacctccatagaagacaccgggaccgatccagcctccgcggccgggaacggtgcattggaacgcggattccccgtgccaagagtgacgtaagtaccgcagtcaccgtccttgacacgggatccgccaccatggaagacgccaaaaacataaagaaaggcccggcgccattctatccgctggaagatggaaccgctggagagcaactgcataaggctatgaagagatacgccctggttcctggaacaattgcttttacagatgcacatatcgaggtggacatcacttacgctgagtacttcgaaatgtccgttcggttggcagaagctatgaaacgatatgggctgaatacaaatcacagaatcgtcgtatgcagtgaaaactctcttcaattctttatgccggtgttgggcgcgttatttatcggagttgcagttgcgcccgcgaacgacatttataatgaacgtgaattgctcaacagtatgggcatttcgcagcctaccgtggtgttcgtttccaaaaaggggttgcaaaaaattttgaacgtgcaaaaaaagctcccaatcatccaaaaaattattatcatggattctaaaacggattaccagggatttcagtcgatgtacacgttcgtcacatctcatctacctcccggttttaatgaatacgattttgtgccagagtccttcgatagggacaagacaattgcactgatcatgaactcctctggatctactggtctgcctaaaggtgtcgctctgcctcatagaactgcctgcgtgagattctcgcatgccagagatcctatttttggcaatcaaatcattccggatactgcgattttaagtgttgttccattccatcacggttttggaatgtttactacactcggatatttgatatgtggatttcgagtcgtcttaatgtatagatttgaagaagagctgtttctgaggagccttcaggattacaagattcaaagtgcgctgctggtgccaaccctattctccttcttcgccaaaagcactctgattgacaaatacgatttatctaatttacacgaaattgcttctggtggcgctcccctctctaaggaagtcggggaagcggttgccaagaggttccatctgccaggtatcaggcaaggatatgggctcactgagactacatcagctattctgattacacccgagggggatgataaaccgggcgcggtcggtaaagttgttccattttttgaagcgaaggttgtggatctggataccgggaaaacgctgggcgttaatcaaagaggcgaactgtgtgtgagaggtcctatgattatgtccggttatgtaaacaatccggaagcgaccaacgccttgattgacaaggatggatggctacattctggagacatagcttactgggacgaagacgaacacttcttcatcgttgaccgcctgaagtctctgattaagtacaaaggctatcaggtggctcccgctgaattggaatccatcttgctccaacaccccaacatcttcgacgcaggtgtcgcaggtcttcccgacgatgacgccggtgaacttcccgccgccgttgttgttttggagcacggaaagacgatgacggaaaaagagatcgtggattacgtcgccagtcaagtaacaaccgcgaaaaagttgcgcggaggagttgtgtttgtggacgaagtaccgaaaggtcttaccggaaaactcgacgcaagaaaaatcagagagatcctcataaaggccaagaagggcggaaagatcgccgtgtaaggtacccgatcagattctagagggccctattctatagtgtcacctaaatgctagagctcgctgatcagcctcgactgtgccttctagttgccagccatctgttgtttgcccctcccccgtgccttccttgaccctggaaggtgccactcccactgtcctttcctaataaaatgaggaaattgcatcgcattgtctgagtaggtgtcattctattctggggggtggggtggggcaggacagcaagggggaggattgggaagacaatagcaggcatgctggggatgcggtgggctctatggcttctgaggcggaaagaaccagctggggctctagggggtatccccacgcgccctgtagcggcgcattaagcgcggcgggtgtggtggttacgcgcagcgtgaccgctacacttgccagcgccctagcgcccgctcctttcgctttcttcccttcctttctcgccacgttcgccggctttccccgtcaagctctaaatcgggggctccctttagggttccgatttagtgctttacggcacctcgaccccaaaaaacttgattagggtgatggttcacgtagtgggccatcgccctgatagacggtttttcgccctttgacgttggagtccacgttctttaatagtggactcttgttccaaactggaacaacactcaaccctatctcggtctattcttttgatttataagggattttgccgatttcggcctattggttaaaaaatgagctgatttaacaaaaatttaacgcgaattaattctgtggaatgtgtgtcagttagggtgtggaaagtccccaggctccccagcaggcagaagtatgcaaagcatgcatctcaattagtcagcaaccaggtgtggaaagtccccaggctccccagcaggcagaagtatgcaaagcatgcatctcaattagtcagcaaccatagtcccgcccctaactccgcccatcccgcccctaactccgcccagttccgcccattctccgccccatggctgactaattttttttatttatgcagaggccgaggccgcctctgcctctgagctattccagaagtagtgaggaggcttttttggaggcctaggcttttgcaaaaagctcccgggagcttgtatatccattttcggatctgatcaagagacaggatgaggatcgtttcgcatgattgaacaagatggattgcacgcaggttctccggccgcttgggtggagaggctattcggctatgactgggcacaacagacaatcggctgctctgatgccgccgtgttccggctgtcagcgcaggggcgcccggttctttttgtcaagaccgacctgtccggtgccctgaatgaactgcaggacgaggcagcgcggctatcgtggctggccacgacgggcgttccttgcgcagctgtgctcgacgttgtcactgaagcgggaagggactggctgctattgggcgaagtgccggggcaggatctcctgtcatctcaccttgctcctgccgagaaagtatccatcatggctgatgcaatgcggcggctgcatacgcttgatccggctacctgcccattcgaccaccaagcgaaacatcgcatcgagcgagcacgtactcggatggaagccggtcttgtcgatcaggatgatctggacgaagagcatcaggggctcgcgccagccgaactgttcgccaggctcaaggcgcgcatgcccgacggcgaggatctcgtcgtgacccatggcgatgcctgcttgccgaatatcatggtggaaaatggccgcttttctggattcatcgactgtggccggctgggtgtggcggaccgctatcaggacatagcgttggctacccgtgatattgctgaagagcttggcggcgaatgggctgaccgcttcctcgtgctttacggtatcgccgctcccgattcgcagcgcatcgccttctatcgccttcttgacgagttcttctgagcgggactctggggttcgaaatgaccgaccaagcgacgcccaacctgccatcacgagatttcgattccaccgccgccttctatgaaaggttgggcttcggaatcgttttccgggacgccggctggatgatcctccagcgcggggatctcatgctggagttcttcgcccaccccaacttgtttattgcagcttataatggttacaaataaagcaatagcatcacaaatttcacaaataaagcatttttttcactgcattctagttgtggtttgtccaaactcatcaatgtatcttatcatgtctgtataccgtcgacctctagctagagcttggcgtaatcatggtcatagctgtttcctgtgtgaaattgttatccgctcacaattccacacaacatacgagccggaagcataaagtgtaaagcctggggtgcctaatgagtgagctaactcacattaattgcgttgcgctcactgcccgctttccagtcgggaaacctgtcgtgccagctgcattaatgaatcggccaacgcgcggggagaggcggtttgcgtattgggcgctcttccgcttcctcgctcactgactcgctgcgctcggtcgttcggctgcggcgagcggtatcagctcactcaaaggcggtaatacggttatccacagaatcaggggataacgcaggaaagaacatgtgagcaaaaggccagcaaaaggccaggaaccgtaaaaaggccgcgttgctggcgtttttccataggctccgcccccctgacgagcatcacaaaaatcgacgctcaagtcagaggtggcgaaacccgacaggactataaagataccaggcgtttccccctggaagctccctcgtgcgctctcctgttccgaccctgccgcttaccggatacctgtccgcctttctcccttcgggaagcgtggcgctttctcatagctcacgctgtaggtatctcagttcggtgtaggtcgttcgctccaagctgggctgtgtgcacgaaccccccgttcagcccgaccgctgcgccttatccggtaactatcgtcttgagtccaacccggtaagacacgacttatcgccactggcagcagccactggtaacaggattagcagagcgaggtatgtaggcggtgctacagagttcttgaagtggtggcctaactacggctacactagaagaacagtatttggtatctgcgctctgctgaagccagttaccttcggaaaaagagttggtagctcttgatccggcaaacaaaccaccgctggtagcggtggtttttttgtttgcaagcagcagattacgcgcagaaaaaaaggatctcaagaagatcctttgatcttttctacggggtctgacgctcagtggaacgaaaactcacgttaagggattttggtcatgagattatcaaaaaggatcttcacctagatccttttaaattaaaaatgaagttttaaatcaatctaaagtatatatgagtaaacttggtctgacagttaccaatgcttaatcagtgaggcacctatctcagcgatctgtctatttcgttcatccatagttgcctgactccccgtcgtgtagataactacgatacgggagggcttaccatctggccccagtgctgcaatgataccgcgagacccacgctcaccggctccagatttatcagcaataaaccagccagccggaagggccgagcgcagaagtggtcctgcaactttatccgcctccatccagtctattaattgttgccgggaagctagagtaagtagttcgccagttaatagtttgcgcaacgttgttgccattgctacaggcatcgtggtgtcacgctcgtcgtttggtatggcttcattcagctccggttcccaacgatcaaggcgagttacatgatcccccatgttgtgcaaaaaagcggttagctccttcggtcctccgatcgttgtcagaagtaagttggccgcagtgttatcactcatggttatggcagcactgcataattctcttactgtcatgccatccgtaagatgcttttctgtgactggtgagtactcaaccaagtcattctgagaatagtgtatgcggcgaccgagttgctcttgcccggcgtcaatacgggataataccgcgccacatagcagaactttaaaagtgctcatcattggaaaacgttcttcggggcgaaaactctcaaggatcttaccgctgttgagatccagttcgatgtaacccactcgtgcacccaactgatcttcagcatcttttactttcaccagcgtttctgggtgagcaaaaacaggaaggcaaaatgccgcaaaaaagggaataagggcgacacggaaatgttgaatactcatactcttcctttttcaatattattgaagcatttatcagggttattgtctcatgagcggatacatatttgaatgtatttagaaaaataaacaaataggggttccgcgcacatttccccgaaaagtgccacctgacgtc

SEQ ID NO: 4 - DNA, 7287 bp, synthetic construct
  misc_feature 1..7287: note = plasmid
  source 1..7287: mol_type = other DNA
gacggatcgggagatctcccgatcccctatggtgcactctcagtacaatctgctctgatgccgcatagttaagccagtatctgctccctgcttgtgtgttggaggtcgctgagtagtgcgcgagcaaaatttaagctacaacaaggcaaggcttgaccgacaattgcatgaagaatctgcttagggttaggcgttttgcgctgcttcgcgatgtacgggccagatatacgcgttgacattgattattgactagttattaatagtaatcaattacggggtcattagttcatagcccatatatggagttccgcgttacataacttacggtaaatggcccgcctggctgaccgcccaacgacccccgcccattgacgtcaataatgacgtatgttcccatagtaacgccaatagggactttccattgacgtcaatgggtggagtatttacggtaaactgcccacttggcagtacatcaagtgtatcatatgccaagtacgccccctattgacgtcaatgacggtaaatggcccgcctggcattatgcccagtacatgaccttatgggactttcctacttggcagtacatctacgtattagtcatcgctattaccatggtgatgcggttttggcagtacatcaatgggcgtggatagcggtttgactcacggggatttccaagtctccaccccattgacgtcaatgggagtttgttttggcaccaaaatcaacgggactttccaaaatgtcgtaacaactccgccccattgacgcaaatgggcggtaggcgtgtacggtgggaggtctatataagcagagctctctggctaactagagaacccactgcttactggcttatcgaaattaatacgactcactatagggaaagctttaatacgactcactataggacagatcgcctggagacgccatccacgctgttttgacctccatagaagacaccgggaccgatccagcctccgcggccgggaacggtgcattggaacgcggattccccgtgccaagagtgacgtaagtaccgcagtcaccgtccttgacacgggatccgccaccatggaagacgccaaaaacataaagaaaggcccggcgccattctatccgctggaagatggaaccgctggagagcaactgcataaggctatgaagagatacgccctggttcctggaacaattgcttttacagatgcacatatcgaggtggacatcacttacgctgagtacttcgaaatgtccgttcggttggcagaagctatgaaacgatatgggctgaatacaaatcacagaatcgtcgtatgcagtgaaaactctcttcaattctttatgccggtgttgggcgcgttatttatcggagttgcagttgcgcccgcgaacgacatttataatgaacgtgaattgctcaacagtatgggcatttcgcagcctaccgtggtgttcgtttccaaaaaggggttgcaaaaaattttgaacgtgcaaaaaaagctcccaatcatccaaaaaattattatcatggattctaaaacggattaccagggatttcagtcgatgtacacgttcgtcacatctcatctacctcccggttttaatgaatacgattttgtgccagagtccttcgatagggacaagacaattgcactgatcatgaactcctctggatctactggtctgcctaaaggtgtcgctctgcctcatagaactgcctgcgtgagattctcgcatgccagagatcctatttttggcaatcaaatcattccggatactgcgattttaagtgttgttccattccatcacggttttggaatgtttactacactcggatatttgatatgtggatttcgagtcgtcttaatgtatagatttgaagaagagctgtttctgaggagccttcaggattacaagattcaaagtgcgctgctggtgccaaccctattctccttcttcgccaaaagcactctgattgacaaatacgatttatctaatttacacgaaattgcttctggtggcgctcccctctctaaggaagtcggggaagcggttgccaagaggttccatctgccaggtatcaggcaaggatatgggctcactgagactacatcagctattctgattacacccgagggggatgataaaccgggcgcggtcggtaaagttgttccattttttgaagcgaaggttgtggatctggataccgggaaaacgctgggcgttaatcaaagaggcgaactgtgtgtgagaggtcctatgattatgtccggttatgtaaacaatccggaagcgaccaacgccttgattgacaaggatggatggctacattctggagacatagcttactgggacgaagacgaacacttcttcatcgttgaccgcctgaagtctctgattaagtacaaaggctatcaggtggctcccgctgaattggaatccatcttgctccaacaccccaacatcttcgacgcaggtgtcgcaggtcttcccgacgatgacgccggtgaacttcccgccgccgttgttgttttggagcacggaaagacgatgacggaaaaagagatcgtggattacgtcgccagtcaagtaacaaccgcgaaaaagttgcgcggaggagttgtgtttgtggacgaagtaccgaaaggtcttaccggaaaactcgacgcaagaaaaatcagagagatcctcataaaggccaagaagggcggaaagatcgccgtgtaaggtacccgggtggcatccctgtgacccctccccagtgcctctcctggccctggaagttgccactccagtgcccaccagccttgtcctaataaaattaagttgcatcgggccctattctatagtgtcacctaaatgctagagctcgctgatcagcctcgactgtgccttctagttgccagccatctgttgtttgcccctcccccgtgccttccttgaccctggaaggtgccactcccactgtcctttcctaataaaatgaggaaattgcatcgcattgtctgagtaggtgtcattctattctggggggtggggtggggcaggacagcaagggggaggattgggaagacaatagcaggcatgctggggatgcggtgggctctatggcttctgaggcggaaagaaccagctggggctctagggggtatccccacgcgccctgtagcggcgcattaagcgcggcgggtgtggtggttacgcgcagcgtgaccgctacacttgccagcgccctagcgcccgctcctttcgctttcttcccttcctttctcgccacgttcgccggctttccccgtcaagctctaaatcgggggctccctttagggttccgatttagtgctttacggcacctcgaccccaaaaaacttgattagggtgatggttcacgtagtgggccatcgccctgatagacggtttttcgccctttgacgttggagtccacgttctttaatagtggactcttgttccaaactggaacaacactcaaccctatctcggtctattcttttgatttataagggattttgccgatttcggcctattggttaaaaaatgagctgatttaacaaaaatttaacgcgaattaattctgtggaatgtgtgtcagttagggtgtggaaagtccccaggctccccagcaggcagaagtatgcaaagcatgcatctcaattagtcagcaaccaggtgtggaaagtccccaggctccccagcaggcagaagtatgcaaagcatgcatctcaattagtcagcaaccatagtcccgcccctaactccgcccatcccgcccctaactccgcccagttccgcccattctccgccccatggctgactaattttttttatttatgcagaggccgaggccgcctctgcctctgagctattccagaagtagtgaggaggcttttttggaggcctaggcttttgcaaaaagctcccgggagcttgtatatccattttcggatctgatcaagagacaggatgaggatcgtttcgcatgattgaacaagatggattgcacgcaggttctccggccgcttgggtggagaggctattcggctatgactgggcacaacagacaatcggctgctctgatgccgccgtgttccggctgtcagcgcaggggcgcccggttctttttgtcaagaccgacctgtccggtgccctgaatgaactgcaggacgaggcagcgcggctatcgtggctggccacgacgggcgttccttgcgcagctgtgctcgacgttgtcactgaagcgggaagggactggctgctattgggcgaagtgccggggcaggatctcctgtcatctcaccttgctcctgccgagaaagtatccatcatggctgatgcaatgcggcggctgcatacgcttgatccggctacctgcccattcgaccaccaagcgaaacatcgcatcgagcgagcacgtactcggatggaagccggtcttgtcgatcaggatgatctggacgaagagcatcaggggctcgcgccagccgaactgttcgccaggctcaaggcgcgcatgcccgacggcgaggatctcgtcgtgacccatggcgatgcctgcttgccgaatatcatggtggaaaatggccgcttttctggattcatcgactgtggccggctgggtgtggcggaccgctatcaggacatagcgttggctacccgtgatattgctgaagagcttggcggcgaatgggctgaccgcttcctcgtgctttacggtatcgccgctcccgattcgcagcgcatcgccttctatcgccttcttgacgagttcttctgagcgggactctggggttcgaaatgaccgaccaagcgacgcccaacctgccatcacgagatttcgattccaccgccgccttctatgaaaggttgggcttcggaatcgttttccgggacgccggctggatgatcctccagcgcggggatctcatgctggagttcttcgcccaccccaacttgtttattgcagcttataatggttacaaataaagcaatagcatcacaaatttcacaaataaagcatttttttcactgcattctagttgtggtttgtccaaactcatcaatgtatcttatcatgtctgtataccgtcgacctctagctagagcttggcgtaatcatggtcatagctgtttcctgtgtgaaattgttatccgctcacaattccacacaacatacgagccggaagcataaagtgtaaagcctggggtgcctaatgagtgagctaactcacattaattgcgttgcgctcactgcccgctttccagtcgggaaacctgtcgtgccagctgcattaatgaatcggccaacgcgcggggagaggcggtttgcgtattgggcgctcttccgcttcctcgctcactgactcgctgcgctcggtcgttcggctgcggcgagcggtatcagctcactcaaaggcggtaatacggttatccacagaatcaggggataacgcaggaaagaacatgtgagcaaaaggccagcaaaaggccaggaaccgtaaaaaggccgcgttgctggcgtttttccataggctccgcccccctgacgagcatcacaaaaatcgacgctcaagtcagaggtggcgaaacccgacaggactataaagataccaggcgtttccccctggaagctccctcgtgcgctctcctgttccgaccctgccgcttaccggatacctgtccgcctttctcccttcgggaagcgtggcgctttctcatagctcacgctgtaggtatctcagttcggtgtaggtcgttcgctccaagctgggctgtgtgcacgaaccccccgttcagcccgaccgctgcgccttatccggtaactatcgtcttgagtccaacccggtaagacacgacttatcgccactggcagcagccactggtaacaggattagcagagcgaggtatgtaggcggtgctacagagttcttgaagtggtggcctaactacggctacactagaagaacagtatttggtatctgcgctctgctgaagccagttaccttcggaaaaagagttggtagctcttgatccggcaaacaaaccaccgctggtagcggtggtttttttgtttgcaagcagcagattacgcgcagaaaaaaaggatctcaagaagatcctttgatcttttctacggggtctgacgctcagtggaacgaaaactcacgttaagggattttggtcatgagattatcaaaaaggatcttcacctagatccttttaaattaaaaatgaagttttaaatcaatctaaagtatatatgagtaaacttggtctgacagttaccaatgcttaatcagtgaggcacctatctcagcgatctgtctatttcgttcatccatagttgcctgactccccgtcgtgtagataactacgatacgggagggcttaccatctggccccagtgctgcaatgataccgcgagacccacgctcaccggctccagatttatcagcaataaaccagccagccggaagggccgagcgcagaagtggtcctgcaactttatccgcctccatccagtctattaattgttgccgggaagctagagtaagtagttcgccagttaatagtttgcgcaacgttgttgccattgctacaggcatcgtggtgtcacgctcgtcgtttggtatggcttcattcagctccggttcccaacgatcaaggcgagttacatgatcccccatgttgtgcaaaaaagcggttagctccttcggtcctccgatcgttgtcagaagtaagttggccgcagtgttatcactcatggttatggcagcactgcataattctcttactgtcatgccatccgtaagatgcttttctgtgactggtgagtactcaaccaagtcattctgagaatagtgtatgcggcgaccgagttgctcttgcccggcgtcaatacgggataataccgcgccacatagcagaactttaaaagtgctcatcattggaaaacgttcttcggggcgaaaactctcaaggatcttaccgctgttgagatccagttcgatgtaacccactcgtgcacccaactgatcttcagcatcttttactttcaccagcgtttctgggtgagcaaaaacaggaaggcaaaatgccgcaaaaaagggaataagggcgacacggaaatgttgaatactcatactcttcctttttcaatattattgaagcatttatcagggttattgtctcatgagcggatacatatttgaatgtatttagaaaaataaacaaataggggttccgcgcacatttccccgaaaagtgccacctgacgtc

SEQ ID NO: 5 - DNA, 6201 bp, synthetic construct
  misc_feature 1..6201: note = plasmid
  source 1..6201: mol_type = other DNA
gacggatcgggagatctcccgatcccctatggtgcactctcagtacaatctgctctgatgccgcatagttaagccagtatctgctccctgcttgtgtgttggaggtcgctgagtagtgcgcgagcaaaatttaagctacaacaaggcaaggcttgaccgacaattgcatgaagaatctgcttagggttaggcgttttgcgctgcttcgcgatgtacgggccagatatacgcgttgacattgattattgactagttattaatagtaatcaattacggggtcattagttcatagcccatatatggagttccgcgttacataacttacggtaaatggcccgcctggctgaccgcccaacgacccccgcccattgacgtcaataatgacgtatgttcccatagtaacgccaatagggactttccattgacgtcaatgggtggagtatttacggtaaactgcccacttggcagtacatcaagtgtatcatatgccaagtacgccccctattgacgtcaatgacggtaaatggcccgcctggcattatgcccagtacatgaccttatgggactttcctacttggcagtacatctacgtattagtcatcgctattaccatggtgatgcggttttggcagtacatcaatgggcgtggatagcggtttgactcacggggatttccaagtctccaccccattgacgtcaatgggagtttgttttggcaccaaaatcaacgggactttccaaaatgtcgtaacaactccgccccattgacgcaaatgggcggtaggcgtgtacggtgggaggtctatataagcagagctctctggctaactagagaacccactgcttactggcttatcgaaattaatacgactcactatagggaaagcttgatcagaacggatccgccaccatggaagacgccaaaaacataaagaaaggcccggcgccattctatccgctggaagatggaaccgctggagagcaactgcataaggctatgaagagatacgccctggttcctggaacaattgcttttacagatgcacatatcgaggtggacatcacttacgctgagtacttcgaaatgtccgttcggttggcagaagctatgaaacgatatgggctgaatacaaatcacagaatcgtcgtatgcagtgaaaactctcttcaattctttatgccggtgttgggcgcgttatttatcggagttgcagttgcgcccgcgaacgacatttataatgaacgtgaattgctcaacagtatgggcatttcgcagcctaccgtggtgttcgtttccaaaaaggggttgcaaaaaattttgaacgtgcaaaaaaagctcccaatcatccaaaaaattattatcatggattctaaaacggattaccagggatttcagtcgatgtacacgttcgtcacatctcatctacctcccggttttaatgaatacgattttgtgccagagtccttcgatagggacaagacaattgcactgatcatgaactcctctggatctactggtctgcctaaaggtgtcgctctgcctcatagaactgcctgcgtgagattctcgcatgccagagatcctatttttggcaatcaaatcattccggatactgcgattttaagtgttgttccattccatcacggttttggaatgtttactacactcggatatttgatatgtggatttcgagtcgtcttaatgtatagatttgaagaagagctgtttctgaggagccttcaggattacaagattcaaagtgcgctgctggtgccaaccctattctccttcttcgccaaaagcactctgattgacaaatacgatttatctaatttacacgaaattgcttctggtggcgctcccctctctaaggaagtcggggaagcggttgccaagaggttccatctgccaggtatcaggcaaggatatgggctcactgagactacatcagctattctgattacacccgagggggatgataaaccgggcgcggtcggtaaagttgttccattttttgaagcgaaggttgtggatctggataccgggaaaacgctgggcgttaatcaaagaggcgaactgtgtgtgagaggtcctatgattatgtccggttatgtaaacaatccggaagcgaccaacgccttgattgacaaggatggatggctacattctggagacatagcttactgggacgaagacgaacacttcttcatcgttgaccgcctgaagtctctgattaagtacaaaggctatcaggtggctcccgctgaattggaatccatcttgctccaacaccccaacatcttcgacgcaggtgtcgcaggtcttcccgacgatgacgccggtgaacttcccgccgccgttgttgttttggagcacggaaagacgatgacggaaaaagagatcgtggattacgtcgccagtcaagtaacaaccgcgaaaaagttgcgcggaggagttgtgtttgtggacgaagtaccgaaaggtcttaccggaaaactcgacgcaagaaaaatcagagagatcctcataaaggccaagaagggcggaaagatcgccgtgtaaggtacccgatcagattctagagggccctattctatagtgtcacctaaatgctagagctcgctgatcagcctcgactgtgccttctagttgccagccatctgttgtttgcccctcccccgtgccttccttgaccctggaaggtgccactcccactgtcctttcctaataaaatgaggaaattgcatcgcattgtctgagtaggtgtcattctattctggggggtggggtggggcaggacagcaagggggaggattgggaagacaatagcaggcatgctggggatgcggtgggctctatggcttctgaggcggaaagaaccagctggggctctagggggtatccccacgcgccctgtagcggcgcattaagcgcggcgggtgtggtggttacgcgcagcgtgaccgctacacttgccagcgccctagcgcccgctcctttcgctttcttcccttcctttctcgccacgttcgccggctttccccgtcaagctctaaatcgggggctccctttagggttccgatttagtgctttacggcacctcgaccccaaaaaacttgattagggtgatggttcacgtagtgggccatcgccctgatagacggtttttcgccctttgacgttggagtccacgttctttaatagtggactcttgttccaaactggaacaacactcaaccctatctcggtctattcttttgatttataagggattttgccgatttcggcctattggttaaaaaatgagctgatttaacaaaaatttaacgcgaattaattctgtggaatgtgtgtcagttagggtgtggaaagtccccaggctccccagcaggcagaagtatgcaaagcatgcatctcaattagtcagcaaccaggtgtggaaagtccccaggctccccagcaggcagaagtatgcaaagcatgcatctcaattagtcagcaaccatagtcccgcccctaactccgcccatcccgcccctaactccgcccagttccgcccattctccgccccatggctgactaattttttttatttatgcagaggccgaggccgcctctgcctctgagctattccagaagtagtgaggaggcttttttggaggcctaggcttttgcaaaaagctcccgggagcttgtatatccattttcggatctgatcaagagacaggatgaggatcgtttcgcgcgggactctggggttcgaaatgaccgaccaagcgacgcccaacctgccatcacgagatttcgattccaccgccgccttctatgaaaggttgggcttcggaatcgttttccgggacgccggctggatgatcctccagcgcggggatctcatgctggagttcttcgcccaccccaacttgtttattgcagcttataatggttacaaataaagcaatagcatcacaaatttcacaaataaagcatttttttcactgcattctagttgtggtttgtccaaactcatcaatgtatcttatcatgtctgtataccgtcgacctctagctagagcttggcgtaatcatggtcatagctgtttcctgtgtgaaattgttatccgctcacaattccacacaacatacgagccggaagcataaagtgtaaagcctggggtgcctaatgagtgagctaactcacattaattgcgttgcgctcactgcccgctttccagtcgggaaacctgtcgtgccagctgcattaatgaatcggccaacgcgcggggagaggcggtttgcgtattgggcgctcttccgcttcctcgctcactgactcgctgcgctcggtcgttcggctgcggcgagcggtatcagctcactcaaaggcggtaatacggttatccacagaatcaggggataacgcaggaaagaacatgtgagcaaaaggccagcaaaaggccaggaaccgtaaaaaggccgcgttgctggcgtttttccataggctccgcccccctgacgagcatcacaaaaatcgacgctcaagtcagaggtggcgaaacccgacaggactataaagataccaggcgtttccccctggaagctccctcgtgcgctctcctgttccgaccctgccgcttaccggatacctgtccgcctttctcccttcgggaagcgtggcgctttctcatagctcacgctgtaggtatctcagttcggtgtaggtcgttcgctccaagctgggctgtgtgcacgaaccccccgttcagcccgaccgctgcgccttatccggtaactatcgtcttgagtccaacccggtaagacacgacttatcgccactggcagcagccactggtaacaggattagcagagcgaggtatgtaggcggtgctacagagttcttgaagtggtggcctaactacggctacactagaagaacagtatttggtatctgcgctctgctgaagccagttaccttcggaaaaagagttggtagctcttgatccggcaaacaaaccaccgctggtagcggtggtttttttgtttgcaagcagcagattacgcgcagaaaaaaaggatctcaagaagatcctttgatcttttctacggggtctgacgctcagtggaacgaaaactcacgttaagggattttggtcatgagattatcaaaaaggatcttcacctagatccttttaaattaaaaatgaagttttaaatcaatctaaagtatatatgagtaaacttggtctgacagttagaaaaactcatcgagcatcaaatgaaactgcaatttattcatatcaggattatcaataccatatttttgaaaaagccgtttctgtaatgaaggagaaaactcaccgaggcagttccataggatggcaagatcctggtatcggtctgcgattccgactcgtccaacatcaatacaacctattaatttcccctcgtcaaaaataaggttatcaagtgagaaatcaccatgagtgacgactgaatccggtgagaatggcaaaagtttatgcatttctttccagacttgttcaacaggccagccattacgctcgtcatcaaaatcactcgcatcaaccaaaccgttattcattcgtgattgcgcctgagcgagacgaaatacgcgatcgctgttaaaaggacaattacaaacaggaatcgaatgcaaccggcgcaggaacactgccagcgcatcaacaatattttcacctgaatcaggatattcttctaatacctggaatgctgttttcccggggatcgcagtggtgagtaaccatgcatcatcaggagtacggataaaatgcttgatggtcggaagaggcataaattccgtcagccagtttagtctgaccatctcatctgtaacatcattggcaacgctacctttgccatgtttcagaaacaactctggcgcatcgggcttcccatacaatcgatagattgtcgcacctgattgcccgacattatcgcgagcccatttatacccatataaatcagcatccatgttggaatttaatcgcggcctagagcaagacgtttcccgttgaatatggctcatactcttcctttttcaatattattgaagcatttatcagggttattgtctcatgagcggatacatatttgaatgtatttagaaaaataaacaaataggggttccgcgcacatttccccgaaaagtgccacctgacgtc

SEQ ID NO: 6 - DNA, 6316 bp, synthetic construct
  misc_feature 1..6316: note = plasmid
  source 1..6316: mol_type = other DNA
gacggatcgggagatctcccgatcccctatggtgcactctcagtacaatctgctctgatgccgcatagttaagccagtatctgctccctgcttgtgtgttggaggtcgctgagtagtgcgcgagcaaaatttaagctacaacaaggcaaggcttgaccgacaattgcatgaagaatctgcttagggttaggcgttttgcgctgcttcgcgatgtacgggccagatatacgcgttgacattgattattgactagttattaatagtaatcaattacggggtcattagttcatagcccatatatggagttccgcgttacataacttacggtaaatggcccgcctggctgaccgcccaacgacccccgcccattgacgtcaataatgacgtatgttcccatagtaacgccaatagggactttccattgacgtcaatgggtggagtatttacggtaaactgcccacttggcagtacatcaagtgtatcatatgccaagtacgccccctattgacgtcaatgacggtaaatggcccgcctggcattatgcccagtacatgaccttatgggactttcctacttggcagtacatctacgtattagtcatcgctattaccatggtgatgcggttttggcagtacatcaatgggcgtggatagcggtttgactcacggggatttccaagtctccaccccattgacgtcaatgggagtttgttttggcaccaaaatcaacgggactttccaaaatgtcgtaacaactccgccccattgacgcaaatgggcggtaggcgtgtacggtgggaggtctatataagcagagctctctggctaactagagaacccactgcttactggcttatcgaaattaatacgactcactatagggaaagcttgatcagaacggatccgccaccatggaagacgccaaaaacataaagaaaggcccggcgccattctatccgctggaagatggaaccgctggagagcaactgcataaggctatgaagagatacgccctggttcctggaacaattgcttttacagatgcacatatcgaggtggacatcacttacgctgagtacttcgaaatgtccgttcggttggcagaagctatgaaacgatatgggctgaatacaaatcacagaatcgtcgtatgcagtgaaaactctcttcaattctttatgccggtgttgggcgcgttatttatcggagttgcagttgcgcccgcgaacgacatttataatgaacgtgaattgctcaacagtatgggcatttcgcagcctaccgtggtgttcgtttccaaaaaggggttgcaaaaaattttgaacgtgcaaaaaaagctcccaatcatccaaaaaattattatcatggattctaaaacggattaccagggatttcagtcgatgtacacgttcgtcacatctcatctacctcccggttttaatgaatacgattttgtgccagagtccttcgatagggacaagacaattgcactgatcatgaactcctctggatctactggtctgcctaaaggtgtcgctctgcctcatagaactgcctgcgtgagattctcgcatgccagagatcctatttttggcaatcaaatcattccggatactgcgattttaagtgttgttccattccatcacggttttggaatgtttactacactcggatatttgatatgtggatttcgagtcgtcttaatgtatagatttgaagaagagctgtttctgaggagccttcaggattacaagattcaaagtgcgctgctggtgccaaccctattctccttcttcgccaaaagcactctgattgacaaatacgatttatctaatttacacgaaattgcttctggtggcgctcccctctctaaggaagtcggggaagcggttgccaagaggttccatctgccaggtatcaggcaaggatatgggctcactgagactacatcagctattctgattacacccgagggggatgataaaccgggcgcggtcggtaaagttgttccattttttgaagcgaaggttgtggatctggataccgggaaaacgctgggcgttaatcaaagaggcgaactgtgtgtgagaggtcctatgattatgtccggttatgtaaacaatccggaagcgaccaacgccttgattgacaaggatggatggctacattctggagacatagcttactgggacgaagacgaacacttcttcatcgttgaccgcctgaagtctctgattaagtacaaaggctatcaggtggctcccgctgaattggaatccatcttgctccaacaccccaacatcttcgacgcaggtgtcgcaggtcttcccgacgatgacgccggtgaacttcccgccgccgttgttgttttggagcacggaaagacgatgacggaaaaagagatcgtggattacgtcgccagtcaagtaacaaccgcgaaaaagttgcgcggaggagttgtgtttgtggacgaagtaccgaaaggtcttaccggaaaactcgacgcaagaaaaatcagagagatcctcataaaggccaagaagggcggaaagatcgccgtgtaaggtacccgatcagattctagagggcccaaaaaaaaaaaaaaaaaaaaaaaaaaaaaagcatatgactaaaaaaaaaaaaaaaaaaaaaaaaaaaaaaaaaaaaaaaaaaaaaaaaaaaaaaaaaaaaaaaaaaaaaaagagaccgtctatagtgtcacctaaatgctagagctcgctgatcagcctcgactgtgccttctagttgccagccatctgttgtttgcccctcccccgtgccttccttgaccctggaaggtgccactcccactgtcctttcctaataaaatgaggaaattgcatcgcattgtctgagtaggtgtcattctattctggggggtggggtggggcaggacagcaagggggaggattgggaagacaatagcaggcatgctggggatgcggtgggctctatggcttctgaggcggaaagaaccagctggggctctagggggtatccccacgcgccctgtagcggcgcattaagcgcggcgggtgtggtggttacgcgcagcgtgaccgctacacttgccagcgccctagcgcccgctcctttcgctttcttcccttcctttctcgccacgttcgccggctttccccgtcaagctctaaatcgggggctccctttagggttccgatttagtgctttacggcacctcgaccccaaaaaacttgattagggtgatggttcacgtagtgggccatcgccctgatagacggtttttcgccctttgacgttggagtccacgttctttaatagtggactcttgttccaaactggaacaacactcaaccctatctcggtctattcttttgatttataagggattttgccgatttcggcctattggttaaaaaatgagctgatttaacaaaaatttaacgcgaattaattctgtggaatgtgtgtcagttagggtgtggaaagtccccaggctccccagcaggcagaagtatgcaaagcatgcatctcaattagtcagcaaccaggtgtggaaagtccccaggctccccagcaggcagaagtatgcaaagcatgcatctcaattagtcagcaaccatagtcccgcccctaactccgcccatcccgcccctaactccgcccagttccgcccattctccgccccatggctgactaattttttttatttatgcagaggccgaggccgcctctgcctctgagctattccagaagtagtgaggaggcttttttggaggcctaggcttttgcaaaaagctcccgggagcttgtatatccattttcggatctgatcaagagacaggatgaggatcgtttcgcgcgggactctggggttcgaaatgaccgaccaagcgacgcccaacctgccatcacgagatttcgattccaccgccgccttctatgaaaggttgggcttcggaatcgttttccgggacgccggctggatgatcctccagcgcggggatctcatgctggagttcttcgcccaccccaacttgtttattgcagcttataatggttacaaataaagcaatagcatcacaaatttcacaaataaagcatttttttcactgcattctagttgtggtttgtccaaactcatcaatgtatcttatcatgtctgtataccgtcgacctctagctagagcttggcgtaatcatggtcatagctgtttcctgtgtgaaattgttatccgctcacaattccacacaacatacgagccggaagcataaagtgtaaagcctggggtgcctaatgagtgagctaactcacattaattgcgttgcgctcactgcccgctttccagtcgggaaacctgtcgtgccagctgcattaatgaatcggccaacgcgcggggagaggcggtttgcgtattgggcgctcttccgcttcctcgctcactgactcgctgcgctcggtcgttcggctgcggcgagcggtatcagctcactcaaaggcggtaatacggttatccacagaatcaggggataacgcaggaaagaacatgtgagcaaaaggccagcaaaaggccaggaaccgtaaaaaggccgcgttgctggcgtttttccataggctccgcccccctgacgagcatcacaaaaatcgacgctcaagtcagaggtggcgaaacccgacaggactataaagataccaggcgtttccccctggaagctccctcgtgcgctctcctgttccgaccctgccgcttaccggatacctgtccgcctttctcccttcgggaagcgtggcgctttctcatagctcacgctgtaggtatctcagttcggtgtaggtcgttcgctccaagctgggctgtgtgcacgaaccccccgttcagcccgaccgctgcgccttatccggtaactatcgtcttgagtccaacccggtaagacacgacttatcgccactggcagcagccactggtaacaggattagcagagcgaggtatgtaggcggtgctacagagttcttgaagtggtggcctaactacggctacactagaagaacagtatttggtatctgcgctctgctgaagccagttaccttcggaaaaagagttggtagctcttgatccggcaaacaaaccaccgctggtagcggtggtttttttgtttgcaagcagcagattacgcgcagaaaaaaaggatctcaagaagatcctttgatcttttctacggggtctgacgctcagtggaacgaaaactcacgttaagggattttggtcatgagattatcaaaaaggatcttcacctagatccttttaaattaaaaatgaagttttaaatcaatctaaagtatatatgagtaaacttggtctgacagttagaaaaactcatcgagcatcaaatgaaactgcaatttattcatatcaggattatcaataccatatttttgaaaaagccgtttctgtaatgaaggagaaaactcaccgaggcagttccataggatggcaagatcctggtatcggtctgcgattccgactcgtccaacatcaatacaacctattaatttcccctcgtcaaaaataaggttatcaagtgagaaatcaccatgagtgacgactgaatccggtgagaatggcaaaagtttatgcatttctttccagacttgttcaacaggccagccattacgctcgtcatcaaaatcactcgcatcaaccaaaccgttattcattcgtgattgcgcctgagcgagacgaaatacgcgatcgctgttaaaaggacaattacaaacaggaatcgaatgcaaccggcgcaggaacactgccagcgcatcaacaatattttcacctgaatcaggatattcttctaatacctggaatgctgttttcccggggatcgcagtggtgagtaaccatgcatcatcaggagtacggataaaatgcttgatggtcggaagaggcataaattccgtcagccagtttagtctgaccatctcatctgtaacatcattggcaacgctacctttgccatgtttcagaaacaactctggcgcatcgggcttcccatacaatcgatagattgtcgcacctgattgcccgacattatcgcgagcccatttatacccatataaatcagcatccatgttggaatttaatcgcggcctagagcaagacgtttcccgttgaatatggctcatactcttcctttttcaatattattgaagcatttatcagggttattgtctcatgagcggatacatatttgaatgtatttagaaaaataaacaaataggggttccgcgcacatttccccgaaaagtgccacctgacgtc

SEQ ID NO: 7 - DNA, 6562 bp, synthetic construct
  misc_feature 1..6562: note = plasmid
  source 1..6562: mol_type = other DNA
gacggatcgggagatctcccgatcccctatggtgcactctcagtacaatctgctctgatgccgcatagttaagccagtatctgctccctgcttgtgtgttggaggtcgctgagtagtgcgcgagcaaaatttaagctacaacaaggcaaggcttgaccgacaattgcatgaagaatctgcttagggttaggcgttttgcgctgcttcgcgatgtacgggccagatatacgcgttgacattgattattgactagttattaatagtaatcaattacggggtcattagttcatagcccatatatggagttccgcgttacataacttacggtaaatggcccgcctggctgaccgcccaacgacccccgcccattgacgtcaataatgacgtatgttcccatagtaacgccaatagggactttccattgacgtcaatgggtggagtatttacggtaaactgcccacttggcagtacatcaagtgtatcatatgccaagtacgccccctattgacgtcaatgacggtaaatggcccgcctggcattatgcccagtacatgaccttatgggactttcctacttggcagtacatctacgtattagtcatcgctattaccatggtgatgcggttttggcagtacatcaatgggcgtggatagcggtttgactcacggggatttccaagtctccaccccattgacgtcaatgggagtttgttttggcaccaaaatcaacgggactttccaaaatgtcgtaacaactccgccccattgacgcaaatgggcggtaggcgtgtacggtgggaggtctatataagcagagctctctggctaactagagaacccactgcttactggcttatcgaaattaatacgactcactatagggaaagctttaatacgactcactataggacagatcgcctggagacgccatccacgctgttttgacctccatagaagacaccgggaccgatccagcctccgcggccgggaacggtgcattggaacgcggattccccgtgccaagagtgacgtaagtaccgcagtcaccgtccttgacacgggatccgccaccatggaagacgccaaaaacataaagaaaggcccggcgccattctatccgctggaagatggaaccgctggagagcaactgcataaggctatgaagagatacgccctggttcctggaacaattgcttttacagatgcacatatcgaggtggacatcacttacgctgagtacttcgaaatgtccgttcggttggcagaagctatgaaacgatatgggctgaatacaaatcacagaatcgtcgtatgcagtgaaaactctcttcaattctttatgccggtgttgggcgcgttatttatcggagttgcagttgcgcccgcgaacgacatttataatgaacgtgaattgctcaacagtatgggcatttcgcagcctaccgtggtgttcgtttccaaaaaggggttgcaaaaaattttgaacgtgcaaaaaaagctcccaatcatccaaaaaattattatcatggattctaaaacggattaccagggatttcagtcgatgtacacgttcgtcacatctcatctacctcccggttttaatgaatacgattttgtgccagagtccttcgatagggacaagacaattgcactgatcatgaactcctctggatctactggtctgcctaaaggtgtcgctctgcctcatagaactgcctgcgtgagattctcgcatgccagagatcctatttttggcaatcaaatcattccggatactgcgattttaagtgttgttccattccatcacggttttggaatgtttactacactcggatatttgatatgtggatttcgagtcgtcttaatgtatagatttgaagaagagctgtttctgaggagccttcaggattacaagattcaaagtgcgctgctggtgccaaccctattctccttcttcgccaaaagcactctgattgacaaatacgatttatctaatttacacgaaattgcttctggtggcgctcccctctctaaggaagtcggggaagcggttgccaagaggttccatctgccaggtatcaggcaaggatatgggctcactgagactacatcagctattctgattacacccgagggggatgataaaccgggcgcggtcggtaaagttgttccattttttgaagcgaaggttgtggatctggataccgggaaaacgctgggcgttaatcaaagaggcgaactgtgtgtgagaggtcctatgattatgtccggttatgtaaacaatccggaagcgaccaacgccttgattgacaaggatggatggctacattctggagacatagcttactgggacgaagacgaacacttcttcatcgttgaccgcctgaagtctctgattaagtacaaaggctatcaggtggctcccgctgaattggaatccatcttgctccaacaccccaacatcttcgacgcaggtgtcgcaggtcttcccgacgatgacgccggtgaacttcccgccgccgttgttgttttggagcacggaaagacgatgacggaaaaagagatcgtggattacgtcgccagtcaagtaacaaccgcgaaaaagttgcgcggaggagttgtgtttgtggacgaagtaccgaaaggtcttaccggaaaactcgacgcaagaaaaatcagagagatcctcataaaggccaagaagggcggaaagatcgccgtgtaaggtacccgggtggcatccctgtgacccctccccagtgcctctcctggccctggaagttgccactccagtgcccaccagccttgtcctaataaaattaagttgcatcgggcccaaaaaaaaaaaaaaaaaaaaaaaaaaaaaagcatatgactaaaaaaaaaaaaaaaaaaaaaaaaaaaaaaaaaaaaaaaaaaaaaaaaaaaaaaaaaaaaaaaaaaaaaaagagaccgtctatagtgtcacctaaatgctagagctcgctgatcagcctcgactgtgccttctagttgccagccatctgttgtttgcccctcccccgtgccttccttgaccctggaaggtgccactcccactgtcctttcctaataaaatgaggaaattgcatcgcattgtctgagtaggtgtcattctattctggggggtggggtggggcaggacagcaagggggaggattgggaagacaatagcaggcatgctggggatgcggtgggctctatggcttctgaggcggaaagaaccagctggggctctagggggtatccccacgcgccctgtagcggcgcattaagcgcggcgggtgtggtggttacgcgcagcgtgaccgctacacttgccagcgccctagcgcccgctcctttcgctttcttcccttcctttctcgccacgttcgccggctttccccgtcaagctctaaatcgggggctccctttagggttccgatttagtgctttacggcacctcgaccccaaaaaacttgattagggtgatggttcacgtagtgggccatcgccctgatagacggtttttcgccctttgacgttggagtccacgttctttaatagtggactcttgttccaaactggaacaacactcaaccctatctcggtctattcttttgatttataagggattttgccgatttcggcctattggttaaaaaatgagctgatttaacaaaaatttaacgcgaattaattctgtggaatgtgtgtcagttagggtgtggaaagtccccaggctccccagcaggcagaagtatgcaaagcatgcatctcaattagtcagcaaccaggtgtggaaagtccccaggctccccagcaggcagaagtatgcaaagcatgcatctcaattagtcagcaaccatagtcccgcccctaactccgcccatcccgcccctaactccgcccagttccgcccattctccgccccatggctgactaattttttttatttatgcagaggccgaggccgcctctgcctctgagctattccagaagtagtgaggaggcttttttggaggcctaggcttttgcaaaaagctcccgggagcttgtatatccattttcggatctgatcaagagacaggatgaggatcgtttcgcgcgggactctggggttcgaaatgaccgaccaagcgacgcccaacctgccatcacgagatttcgattccaccgccgccttctatgaaaggttgggcttcggaatcgttttccgggacgccggctggatgatcctccagcgcggggatctcatgctggagttcttcgcccaccccaacttgtttattgcagcttataatggttacaaataaagcaatagcatcacaaatttcacaaataaagcatttttttcactgcattctagttgtggtttgtccaaactcatcaatgtatcttatcatgtctgtataccgtcgacctctagctagagcttggcgtaatcatggtcatagctgtttcctgtgtgaaattgttatccgctcacaattccacacaacatacgagccggaagcataaagtgtaaagcctggggtgcctaatgagtgagctaactcacattaattgcgttgcgctcactgcccgctttccagtcgggaaacctgtcgtgccagctgcattaatgaatcggccaacgcgcggggagaggcggtttgcgtattgggcgctcttccgcttcctcgctcactgactcgctgcgctcggtcgttcggctgcggcgagcggtatcagctcactcaaaggcggtaatacggttatccacagaatcaggggataacgcaggaaagaacatgtgagcaaaaggccagcaaaaggccaggaaccgtaaaaaggccgcgttgctggcgtttttccataggctccgcccccctgacgagcatcacaaaaatcgacgctcaagtcagaggtggcgaaacccgacaggactataaagataccaggcgtttccccctggaagctccctcgtgcgctctcctgttccgaccctgccgcttaccggatacctgtccgcctttctcccttcgggaagcgtggcgctttctcatagctcacgctgtaggtatctcagttcggtgtaggtcgttcgctccaagctgggctgtgtgcacgaaccccccgttcagcccgaccgctgcgccttatccggtaactatcgtcttgagtccaacccggtaagacacgacttatcgccactggcagcagccactggtaacaggattagcagagcgaggtatgtaggcggtgctacagagttcttgaagtggtggcctaactacggctacactagaagaacagtatttggtatctgcgctctgctgaagccagttaccttcggaaaaagagttggtagctcttgatccggcaaacaaaccaccgctggtagcggtggtttttttgtttgcaagcagcagattacgcgcagaaaaaaaggatctcaagaagatcctttgatcttttctacggggtctgacgctcagtggaacgaaaactcacgttaagggattttggtcatgagattatcaaaaaggatcttcacctagatccttttaaattaaaaatgaagttttaaatcaatctaaagtatatatgagtaaacttggtctgacagttagaaaaactcatcgagcatcaaatgaaactgcaatttattcatatcaggattatcaataccatatttttgaaaaagccgtttctgtaatgaaggagaaaactcaccgaggcagttccataggatggcaagatcctggtatcggtctgcgattccgactcgtccaacatcaatacaacctattaatttcccctcgtcaaaaataaggttatcaagtgagaaatcaccatgagtgacgactgaatccggtgagaatggcaaaagtttatgcatttctttccagacttgttcaacaggccagccattacgctcgtcatcaaaatcactcgcatcaaccaaaccgttattcattcgtgattgcgcctgagcgagacgaaatacgcgatcgctgttaaaaggacaattacaaacaggaatcgaatgcaaccggcgcaggaacactgccagcgcatcaacaatattttcacctgaatcaggatattcttctaatacctggaatgctgttttcccggggatcgcagtggtgagtaaccatgcatcatcaggagtacggataaaatgcttgatggtcggaagaggcataaattccgtcagccagtttagtctgaccatctcatctgtaacatcattggcaacgctacctttgccatgtttcagaaacaactctggcgcatcgggcttcccatacaatcgatagattgtcgcacctgattgcccgacattatcgcgagcccatttatacccatataaatcagcatccatgttggaatttaatcgcggcctagagcaagacgtttcccgttgaatatggctcatactcttcctttttcaatattattgaagcatttatcagggttattgtctcatgagcggatacatatttgaatgtatttagaaaaataaacaaataggggttccgcgcacatttccccgaaaagtgccacctgacgtc

SEQ ID NO: 8 - DNA, 8728 bp, synthetic construct
  misc_feature 1..8728: note = plasmid
  source 1..8728: mol_type = other DNA
gacggatcgggagatctcccgatcccctatggtgcactctcagtacaatctgctctgatgccgcatagttaagccagtatctgctccctgcttgtgtgttggaggtcgctgagtagtgcgcgagcaaaatttaagctacaacaaggcaaggcttgaccgacaattgcatgaagaatctgcttagggttaggcgttttgcgctgcttcgcgatgtacgggccagatatacgcgttgacattgattattgactagttattaatagtaatcaattacggggtcattagttcatagcccatatatggagttccgcgttacataacttacggtaaatggcccgcctggctgaccgcccaacgacccccgcccattgacgtcaataatgacgtatgttcccatagtaacgccaatagggactttccattgacgtcaatgggtggagtatttacggtaaactgcccacttggcagtacatcaagtgtatcatatgccaagtacgccccctattgacgtcaatgacggtaaatggcccgcctggcattatgcccagtacatgaccttatgggactttcctacttggcagtacatctacgtattagtcatcgctattaccatggtgatgcggttttggcagtacatcaatgggcgtggatagcggtttgactcacggggatttccaagtctccaccccattgacgtcaatgggagtttgttttggcaccaaaatcaacgggactttccaaaatgtcgtaacaactccgccccattgacgcaaatgggcggtaggcgtgtacggtgggaggtctatataagcagagctctctggctaactagagaacccactgcttactggcttatcgaaattaatacgactcactatagggaaagctttaatacgactcactataggacagatcgcctggagacgccatccacgctgttttgacctccatagaagacaccgggaccgatccagcctccgcggccgggaacggtgcattggaacgcggattccccgtgccaagagtgacgtaagtaccgcagtcaccgtccttgacacgggatccgccaccatgttcgtgttcctggtgctgctgcctctggtgtccagccagtgtgtgaacctgaggaccagaacacagctgcctccagcctacaccaacagctttaccagaggcgtgtactaccccgacaaggtgttcagatccagcgtgctgcactctacccaggacctgttcctgcctttcttcagcaacgtgacctggttccacgccatccacgtgtccggcaccaatggcaccaagagattcgacaaccccgtgctgcccttcaacgacggggtgtactttgccagcatcgagaagtccaacatcatcagaggctggatcttcggcaccacactggacagcaagacccagagcctgctgatcgtgaacaacgccaccaacgtggtcatcaaagtgtgcgagttccagttctgcaacgaccccttcctggacgtctactaccacaagaacaacaagagctggatggaaagcggcgtgtacagcagcgccaacaactgcaccttcgagtacgtgtcccagcctttcctgatggacctggaaggcaagcagggcaacttcaagaacctgcgcgagttcgtgtttaagaacatcgacggctacttcaagatctacagcaagcacacccctatcaacctcgtgcgggatctgcctcagggcttctctgctctggaacccctggtggatctgcccatcggcatcaacatcacccggtttcagacactgctggccctgcacagaagctacctgacacctggcgatagcagcagcggactgacagctggtgccgccgcttactatgtgggctacctgcagcctagaaccttcctgctgaagtacaacgagaacggcaccatcaccgacgccgtggattgtgctctggaccctctgagcgagacaaagtgcaccctgaagtccttcaccgtggaaaagggcatctaccagaccagcaacttccgggtgcagcccaccgaatccatcgtgcggttccccaatatcaccaatctgtgccccttcggcgaggtgttcaatgccaccagattcgcctctgtgtacgcctggaaccggaagcggatcagcaattgcgtggccgactactccgtgctgtacaactccgccagcttcagcaccttcaagtgctacggcgtgtcccctaccaagctgaacgacctgtgcttcacaaacgtgtacgccgacagcttcgtgatccggggagatgaagtgcggcagattgcccctggacagacaggcaacatcgccgactacaactacaagctgcccgacgacttcaccggctgtgtgattgcctggaacagcaacaacctggactccaaagtcggcggcaactacaattaccggtacaggctgttccggaagtccaatctgaagcccttcgagcgggacatctccaccgagatctatcaggccggcagcaagccttgtaacggcgtggaaggcttcaactgctacttcccactgcagtcctacggctttcagcccacaaatggcgtgggctatcagccctacagagtggtggtgctgagcttcgaactgctgcatgcccctgccacagtgtgcggccctaagaaaagcaccaatctcgtgaagaacaaatgcgtgaacttcaacttcaacggcctgaccggcaccggcgtgctgacagagagcaacaagaagttcctgccattccagcagtttggccgggatatcgccgataccacagacgccgttagagatccccagacactggaaatcctggacatcaccccttgcagcttcggcggagtgtctgtgatcacccctggcaccaacaccagcaatcaggtggcagtgctgtaccagggcgtgaactgtaccgaagtgcccgtggccattcacgccgatcagctgacacctacatggcgggtgtactccaccggcagcaatgtgtttcagaccagagccggctgtctgatcggagccgagcacgtgaacaatagctacgagtgcgacatccccatcggcgctggaatctgcgccagctaccagacacagacaaacagccggcggagagccagaagcgtggccagccagagcatcattgcctacacaatgtctctgggcgccgagaacagcgtggcctactccaacaactctatcgctatccccaccaacttcaccatcagcgtgaccacagagatcctgcctgtgtccatgaccaagaccagcgtggactgcaccatgtacatctgcggcgattccaccgagtgctccaacctgctgctgcagtacggcagcttctgcacccagctgaatagagccctgacagggatcgccgtggaacaggacaagaacacccaagaggtgttcgcccaagtgaagcagatctacaagacccctcctatcaaggacttcggcggcttcaatttcagccagattctgcccgatcctagcaagcccagcaagcggagcttcatcgaggacctgctgttcaacaaagtgacactggccgacgccggcttcatcaagcagtatggcgattgtctgggcgacattgccgccagggatctgatttgcgcccagaagtttaacggactgacagtgctgcctcctctgctgaccgatgagatgatcgcccagtacacatctgccctgctggccggcacaatcacaagcggctggacatttggagcaggcgccgctctgcagatcccctttgctatgcagatggcctaccggttcaacggcatcggagtgacccagaatgtgctgtacgagaaccagaagctgatcgccaaccagttcaacagcgccatcggcaagatccaggacagcctgagcagcacagcaagcgccctgggaaagctgcagaacgtggtcaaccagaatgcccaggcactgaacaccctggtcaagcagctgtcctccaacttcggcgccatcagctctgtgctgaacgatatcctgagcagactggaccctcctgaggccgaggtgcagatcgacagactgatcacaggcagactgcagagcctccagacatacgtgacccagcagctgatcagagccgccgagattagagcctctgccaatctggccgccaccaagatgtctgagtgtgtgctgggccagagcaagagagtggacttttgcggcaagggctaccacctgatgagcttccctcagtctgcccctcacggcgtggtgtttctgcacgtgacatatgtgcccgctcaagagaagaatttcaccaccgctccagccatctgccacgacggcaaagcccactttcctagagaaggcgtgttcgtgtccaacggcacccattggttcgtgacacagcggaacttctacgagccccagatcatcaccaccgacaacaccttcgtgtctggcaactgcgacgtcgtgatcggcattgtgaacaataccgtgtacgaccctctgcagcccgagctggacagcttcaaagaggaactggacaagtactttaagaaccacacaagccccgacgtggacctgggcgatatcagcggaatcaatgccagcgtcgtgaacatccagaaagagatcgaccggctgaacgaggtggccaagaatctgaacgagagcctgatcgacctgcaagaactggggaagtacgagcagtacatcaagtggccctggtacatctggctgggctttatcgccggactgattgccatcgtgatggtcacaatcatgctgtgttgcatgaccagctgctgtagctgcctgaagggctgttgtagctgtggcagctgctgcaagttcgacgaggacgattctgagcccgtgctgaagggcgtgaaactgcactacacatgatgaggtacccgggtggcatccctgtgacccctccccagtgcctctcctggccctggaagttgccactccagtgcccaccagccttgtcctaataaaattaagttgcatcgggcccaaaaaaaaaaaaaaaaaaaaaaaaaaaaaagcatatgactaaaaaaaaaaaaaaaaaaaaaaaaaaaaaaaaaaaaaaaaaaaaaaaaaaaaaaaaaaaaaaaaaaaaaaagagaccgtctatagtgtcacctaaatgctagagctcgctgatcagcctcgactgtgccttctagttgccagccatctgttgtttgcccctcccccgtgccttccttgaccctggaaggtgccactcccactgtcctttcctaataaaatgaggaaattgcatcgcattgtctgagtaggtgtcattctattctggggggtggggtggggcaggacagcaagggggaggattgggaagacaatagcaggcatgctggggatgcggtgggctctatggcttctgaggcggaaagaaccagctggggctctagggggtatccccacgcgccctgtagcggcgcattaagcgcggcgggtgtggtggttacgcgcagcgtgaccgctacacttgccagcgccctagcgcccgctcctttcgctttcttcccttcctttctcgccacgttcgccggctttccccgtcaagctctaaatcgggggctccctttagggttccgatttagtgctttacggcacctcgaccccaaaaaacttgattagggtgatggttcacgtagtgggccatcgccctgatagacggtttttcgccctttgacgttggagtccacgttctttaatagtggactcttgttccaaactggaacaacactcaaccctatctcggtctattcttttgatttataagggattttgccgatttcggcctattggttaaaaaatgagctgatttaacaaaaatttaacgcgaattaattctgtggaatgtgtgtcagttagggtgtggaaagtccccaggctccccagcaggcagaagtatgcaaagcatgcatctcaattagtcagcaaccaggtgtggaaagtccccaggctccccagcaggcagaagtatgcaaagcatgcatctcaattagtcagcaaccatagtcccgcccctaactccgcccatcccgcccctaactccgcccagttccgcccattctccgccccatggctgactaattttttttatttatgcagaggccgaggccgcctctgcctctgagctattccagaagtagtgaggaggcttttttggaggcctaggcttttgcaaaaagctcccgggagcttgtatatccattttcggatctgatcaagagacaggatgaggatcgtttcgcgcgggactctggggttcgaaatgaccgaccaagcgacgcccaacctgccatcacgagatttcgattccaccgccgccttctatgaaaggttgggcttcggaatcgttttccgggacgccggctggatgatcctccagcgcggggatctcatgctggagttcttcgcccaccccaacttgtttattgcagcttataatggttacaaataaagcaatagcatcacaaatttcacaaataaagcatttttttcactgcattctagttgtggtttgtccaaactcatcaatgtatcttatcatgtctgtataccgtcgacctctagctagagcttggcgtaatcatggtcatagctgtttcctgtgtgaaattgttatccgctcacaattccacacaacatacgagccggaagcataaagtgtaaagcctggggtgcctaatgagtgagctaactcacattaattgcgttgcgctcactgcccgctttccagtcgggaaacctgtcgtgccagctgcattaatgaatcggccaacgcgcggggagaggcggtttgcgtattgggcgctcttccgcttcctcgctcactgactcgctgcgctcggtcgttcggctgcggcgagcggtatcagctcactcaaaggcggtaatacggttatccacagaatcaggggataacgcaggaaagaacatgtgagcaaaaggccagcaaaaggccaggaaccgtaaaaaggccgcgttgctggcgtttttccataggctccgcccccctgacgagcatcacaaaaatcgacgctcaagtcagaggtggcgaaacccgacaggactataaagataccaggcgtttccccctggaagctccctcgtgcgctctcctgttccgaccctgccgcttaccggatacctgtccgcctttctcccttcgggaagcgtggcgctttctcatagctcacgctgtaggtatctcagttcggtgtaggtcgttcgctccaagctgggctgtgtgcacgaaccccccgttcagcccgaccgctgcgccttatccggtaactatcgtcttgagtccaacccggtaagacacgacttatcgccactggcagcagccactggtaacaggattagcagagcgaggtatgtaggcggtgctacagagttcttgaagtggtggcctaactacggctacactagaagaacagtatttggtatctgcgctctgctgaagccagttaccttcggaaaaagagttggtagctcttgatccggcaaacaaaccaccgctggtagcggtggtttttttgtttgcaagcagcagattacgcgcagaaaaaaaggatctcaagaagatcctttgatcttttctacggggtctgacgctcagtggaacgaaaactcacgttaagggattttggtcatgagattatcaaaaaggatcttcacctagatccttttaaattaaaaatgaagttttaaatcaatctaaagtatatatgagtaaacttggtctgacagttagaaaaactcatcgagcatcaaatgaaactgcaatttattcatatcaggattatcaataccatatttttgaaaaagccgtttctgtaatgaaggagaaaactcaccgaggcagttccataggatggcaagatcctggtatcggtctgcgattccgactcgtccaacatcaatacaacctattaatttcccctcgtcaaaaataaggttatcaagtgagaaatcaccatgagtgacgactgaatccggtgagaatggcaaaagtttatgcatttctttccagacttgttcaacaggccagccattacgctcgtcatcaaaatcactcgcatcaaccaaaccgttattcattcgtgattgcgcctgagcgagacgaaatacgcgatcgctgttaaaaggacaattacaaacaggaatcgaatgcaaccggcgcaggaacactgccagcgcatcaacaatattttcacctgaatcaggatattcttctaatacctggaatgctgttttcccggggatcgcagtggtgagtaaccatgcatcatcaggagtacggataaaatgcttgatggtcggaagaggcataaattccgtcagccagtttagtctgaccatctcatctgtaacatcattggcaacgctacctttgccatgtttcagaaacaactctggcgcatcgggcttcccatacaatcgatagattgtcgcacctgattgcccgacattatcgcgagcccatttatacccatataaatcagcatccatgttggaatttaatcgcggcctagagcaagacgtttcccgttgaatatggctcatactcttcctttttcaatattattgaagcatttatcagggttattgtctcatgagcggatacatatttgaatgtatttagaaaaataaacaaataggggttccgcgcacatttccccgaaaagtgccacctgacgtc

SEQ ID NO: 9 - DNA, 170 bp, synthetic construct
  misc_feature 1..170: note = 5'UTR
  source 1..170: mol_type = other DNA
taatacgactcactataggacagatcgcctggagacgccatccacgctgttttgacctccatagaagacaccgggaccgatccagcctccgcggccgggaacggtgcattggaacgcggattccccgtgccaagagtgacgtaagtaccgcagtcaccgtccttgacacg

SEQ ID NO: 10 - DNA, 100 bp, synthetic construct
  misc_feature 1..100: note = 3'UTR
  source 1..100: mol_type = other DNA
cgggtggcatccctgtgacccctccccagtgcctctcctggccctggaagttgccactccagtgcccaccagccttgtcctaataaaattaagttgcatc

SEQ ID NO: 11 - DNA, 110 bp, synthetic construct
  misc_feature 1..110: note = polyA
  source 1..110: mol_type = other DNA
aaaaaaaaaaaaaaaaaaaaaaaaaaaaaagcatatgactaaaaaaaaaaaaaaaaaaaaaaaaaaaaaaaaaaaaaaaaaaaaaaaaaaaaaaaaaaaaaaaaaaaaaa

SEQ ID NO: 12 - DNA, 3819 bp, synthetic construct
  misc_feature 1..3819: note = DNA
  source 1..3819: mol_type = other DNA
atgttcgtgttcctggtgctgctgcctctggtgtccagccagtgtgtgaacctgaggaccagaacacagctgcctccagcctacaccaacagctttaccagaggcgtgtactaccccgacaaggtgttcagatccagcgtgctgcactctacccaggacctgttcctgcctttcttcagcaacgtgacctggttccacgccatccacgtgtccggcaccaatggcaccaagagattcgacaaccccgtgctgcccttcaacgacggggtgtactttgccagcatcgagaagtccaacatcatcagaggctggatcttcggcaccacactggacagcaagacccagagcctgctgatcgtgaacaacgccaccaacgtggtcatcaaagtgtgcgagttccagttctgcaacgaccccttcctggacgtctactaccacaagaacaacaagagctggatggaaagcggcgtgtacagcagcgccaacaactgcaccttcgagtacgtgtcccagcctttcctgatggacctggaaggcaagcagggcaacttcaagaacctgcgcgagttcgtgtttaagaacatcgacggctacttcaagatctacagcaagcacacccctatcaacctcgtgcgggatctgcctcagggcttctctgctctggaacccctggtggatctgcccatcggcatcaacatcacccggtttcagacactgctggccctgcacagaagctacctgacacctggcgatagcagcagcggactgacagctggtgccgccgcttactatgtgggctacctgcagcctagaaccttcctgctgaagtacaacgagaacggcaccatcaccgacgccgtggattgtgctctggaccctctgagcgagacaaagtgcaccctgaagtccttcaccgtggaaaagggcatctaccagaccagcaacttccgggtgcagcccaccgaatccatcgtgcggttccccaatatcaccaatctgtgccccttcggcgaggtgttcaatgccaccagattcgcctctgtgtacgcctggaaccggaagcggatcagcaattgcgtggccgactactccgtgctgtacaactccgccagcttcagcaccttcaagtgctacggcgtgtcccctaccaagctgaacgacctgtgcttcacaaacgtgtacgccgacagcttcgtgatccggggagatgaagtgcggcagattgcccctggacagacaggcaacatcgccgactacaactacaagctgcccgacgacttcaccggctgtgtgattgcctggaacagcaacaacctggactccaaagtcggcggcaactacaattaccggtacaggctgttccggaagtccaatctgaagcccttcgagcgggacatctccaccgagatctatcaggccggcagcaagccttgtaacggcgtggaaggcttcaactgctacttcccactgcagtcctacggctttcagcccacaaatggcgtgggctatcagccctacagagtggtggtgctgagcttcgaactgctgcatgcccctgccacagtgtgcggccctaagaaaagcaccaatctcgtgaagaacaaatgcgtgaacttcaacttcaacggcctgaccggcaccggcgtgctgacagagagcaacaagaagttcctgccattccagcagtttggccgggatatcgccgataccacagacgccgttagagatccccagacactggaaatcctggacatcaccccttgcagcttcggcggagtgtctgtgatcacccctggcaccaacaccagcaatcaggtggcagtgctgtaccagggcgtgaactgtaccgaagtgcccgtggccattcacgccgatcagctgacacctacatggcgggtgtactccaccggcagcaatgtgtttcagaccagagccggctgtctgatcggagccgagcacgtgaacaatagctacgagtgcgacatccccatcggcgctggaatctgcgccagctaccagacacagacaaacagccggcggagagccagaagcgtggccagccagagcatcattgcctacacaatgtctctgggcgccgagaacagcgtggcctactccaacaactctatcgctatccccaccaacttcaccatcagcgtgaccacagagatcctgcctgtgtccatgaccaagaccagcgtggactgcaccatgtacatctgcggcgattccaccgagtgctccaacctgctgctgcagtacggcagcttctgcacccagctgaatagagccctgacagggatcgccgtggaacaggacaagaacacccaagaggtgttcgcccaagtgaagcagatctacaagacccctcctatcaaggacttcggcggcttcaatttcagccagattctgcccgatcctagcaagcccagcaagcggagcttcatcgaggacctgctgttcaacaaagtgacactggccgacgccggcttcatcaagcagtatggcgattgtctgggcgacattgccgccagggatctgatttgcgcccagaagtttaacggactgacagtgctgcctcctctgctgaccgatgagatgatcgcccagtacacatctgccctgctggccggcacaatcacaagcggctggacatttggagcaggcgccgctctgcagatcccctttgctatgcagatggcctaccggttcaacggcatcggagtgacccagaatgtgctgtacgagaaccagaagctgatcgccaaccagttcaacagcgccatcggcaagatccaggacagcctgagcagcacagcaagcgccctgggaaagctgcagaacgtggtcaaccagaatgcccaggcactgaacaccctggtcaagcagctgtcctccaacttcggcgccatcagctctgtgctgaacgatatcctgagcagactggaccctcctgaggccgaggtgcagatcgacagactgatcacaggcagactgcagagcctccagacatacgtgacccagcagctgatcagagccgccgagattagagcctctgccaatctggccgccaccaagatgtctgagtgtgtgctgggccagagcaagagagtggacttttgcggcaagggctaccacctgatgagcttccctcagtctgcccctcacggcgtggtgtttctgcacgtgacatatgtgcccgctcaagagaagaatttcaccaccgctccagccatctgccacgacggcaaagcccactttcctagagaaggcgtgttcgtgtccaacggcacccattggttcgtgacacagcggaacttctacgagccccagatcatcaccaccgacaacaccttcgtgtctggcaactgcgacgtcgtgatcggcattgtgaacaataccgtgtacgaccctctgcagcccgagctggacagcttcaaagaggaactggacaagtactttaagaaccacacaagccccgacgtggacctgggcgatatcagcggaatcaatgccagcgtcgtgaacatccagaaagagatcgaccggctgaacgaggtggccaagaatctgaacgagagcctgatcgacctgcaagaactggggaagtacgagcagtacatcaagtggccctggtacatctggctgggctttatcgccggactgattgccatcgtgatggtcacaatcatgctgtgttgcatgaccagctgctgtagctgcctgaagggctgttgtagctgtggcagctgctgcaagttcgacgaggacgattctgagcccgtgctgaagggcgtgaaactgcactacacatgatga

SEQ ID NO: 13 - protein, 1271 aa, synthetic construct
  REGION 1..1271: note = AA sequence
MFVFLVLLPLVSSQCVNLRTRTQLPPAYTNSFTRGVYYPDKVFRSSVLHSTQDLFLPFFSNVTWFHAIHVSGTNGTKRFDNPVLPFNDGVYFASIEKSNIIRGWIFGTTLDSKTQSLLIVNNATNVVIKVCEFQFCNDPFLDVYYHKNNKSWMESGVYSSANNCTFEYVSQPFLMDLEGKQGNFKNLREFVFKNIDGYFKIYSKHTPINLVRDLPQGFSALEPLVDLPIGINITRFQTLLALHRSYLTPGDSSSGLTAGAAAYYVGYLQPRTFLLKYNENGTITDAVDCALDPLSETKCTLKSFTVEKGIYQTSNFRVQPTESIVRFPNITNLCPFGEVFNATRFASVYAWNRKRISNCVADYSVLYNSASFSTFKCYGVSPTKLNDLCFTNVYADSFVIRGDEVRQIAPGQTGNIADYNYKLPDDFTGCVIAWNSNNLDSKVGGNYNYRYRLFRKSNLKPFERDISTEIYQAGSKPCNGVEGFNCYFPLQSYGFQPTNGVGYQPYRVVVLSFELLHAPATVCGPKKSTNLVKNKCVNFNFNGLTGTGVLTESNKKFLPFQQFGRDIADTTDAVRDPQTLEILDITPCSFGGVSVITPGTNTSNQVAVLYQGVNCTEVPVAIHADQLTPTWRVYSTGSNVFQTRAGCLIGAEHVNNSYECDIPIGAGICASYQTQTNSRRRARSVASQSIIAYTMSLGAENSVAYSNNSIAIPTNFTISVTTEILPVSMTKTSVDCTMYICGDSTECSNLLLQYGSFCTQLNRALTGIAVEQDKNTQEVFAQVKQIYKTPPIKDFGGFNFSQILPDPSKPSKRSFIEDLLFNKVTLADAGFIKQYGDCLGDIAARDLICAQKFNGLTVLPPLLTDEMIAQYTSALLAGTITSGWTFGAGAALQIPFAMQMAYRFNGIGVTQNVLYENQKLIANQFNSAIGKIQDSLSSTASALGKLQNVVNQNAQALNTLVKQLSSNFGAISSVLNDILSRLDPPEAEVQIDRLITGRLQSLQTYVTQQLIRAAEIRASANLAATKMSECVLGQSKRVDFCGKGYHLMSFPQSAPHGVVFLHVTYVPAQEKNFTTAPAICHDGKAHFPREGVFVSNGTHWFVTQRNFYEPQIITTDNTFVSGNCDVVIGIVNNTVYDPLQPELDSFKEELDKYFKNHTSPDVDLGDISGINASVVNIQKEIDRLNEVAKNLNESLIDLQELGKYEQYIKWPWYIWLGFIAGLIAIVMVTIMLCCMTSCCSCLKGCCSCGSCCKFDEDDSEPVLKGVKLHYT

SEQ ID NO: 14 - RNA, 3819 nt, synthetic construct
  misc_feature 1..3819: note = RNA
  source 1..3819: mol_type = other RNA
atgttcgtgttcctggtgctgctgcctctggtgtccagccagtgtgtgaacctgaggaccagaacacagctgcctccagcctacaccaacagctttaccagaggcgtgtactaccccgacaaggtgttcagatccagcgtgctgcactctacccaggacctgttcctgcctttcttcagcaacgtgacctggttccacgccatccacgtgtccggcaccaatggcaccaagagattcgacaaccccgtgctgcccttcaacgacggggtgtactttgccagcatcgagaagtccaacatcatcagaggctggatcttcggcaccacactggacagcaagacccagagcctgctgatcgtgaacaacgccaccaacgtggtcatcaaagtgtgcgagttccagttctgcaacgaccccttcctggacgtctactaccacaagaacaacaagagctggatggaaagcggcgtgtacagcagcgccaacaactgcaccttcgagtacgtgtcccagcctttcctgatggacctggaaggcaagcagggcaacttcaagaacctgcgcgagttcgtgtttaagaacatcgacggctacttcaagatctacagcaagcacacccctatcaacctcgtgcgggatctgcctcagggcttctctgctctggaacccctggtggatctgcccatcggcatcaacatcacccggtttcagacactgctggccctgcacagaagctacctgacacctggcgatagcagcagcggactgacagctggtgccgccgcttactatgtgggctacctgcagcctagaaccttcctgctgaagtacaacgagaacggcaccatcaccgacgccgtggattgtgctctggaccctctgagcgagacaaagtgcaccctgaagtccttcaccgtggaaaagggcatctaccagaccagcaacttccgggtgcagcccaccgaatccatcgtgcggttccccaatatcaccaatctgtgccccttcggcgaggtgttcaatgccaccagattcgcctctgtgtacgcctggaaccggaagcggatcagcaattgcgtggccgactactccgtgctgtacaactccgccagcttcagcaccttcaagtgctacggcgtgtcccctaccaagctgaacgacctgtgcttcacaaacgtgtacgccgacagcttcgtgatccggggagatgaagtgcggcagattgcccctggacagacaggcaacatcgccgactacaactacaagctgcccgacgacttcaccggctgtgtgattgcctggaacagcaacaacctggactccaaagtcggcggcaactacaattaccggtacaggctgttccggaagtccaatctgaagcccttcgagcgggacatctccaccgagatctatcaggccggcagcaagccttgtaacggcgtggaaggcttcaactgctacttcccactgcagtcctacggctttcagcccacaaatggcgtgggctatcagccctacagagtggtggtgctgagcttcgaactgctgcatgcccctgccacagtgtgcggccctaagaaaagcaccaatctcgtgaagaacaaatgcgtgaacttcaacttcaacggcctgaccggcaccggcgtgctgacagagagcaacaagaagttcctgccattccagcagtttggccgggatatcgccgataccacagacgccgttagagatccccagacactggaaatcctggacatcaccccttgcagcttcggcggagtgtctgtgatcacccctggcaccaacaccagcaatcaggtggcagtgctgtaccagggcgtgaactgtaccgaagtgcccgtggccattcacgccgatcagctgacacctacatggcgggtgtactccaccggcagcaatgtgtttcagaccagagccggctgtctgatcggagccgagcacgtgaacaatagctacgagtgcgacatccccatcggcgctggaatctgcgccagctaccagacacagacaaacagccggcggagagccagaagcgtggccagccagagcatcattgcctacacaatgtctctgggcgccgagaacagcgtggcctactccaacaactctatcgctatccccaccaacttcaccatcagcgtgaccacagagatcctgcctgtgtccatgaccaagaccagcgtggactgcaccatgtacatctgcggcgattccaccgagtgctccaacctgctgctgcagtacggcagcttctgcacccagctgaatagagccctgacagggatcgccgtggaacaggacaagaacacccaagaggtgttcgcccaagtgaagcagatctacaagacccctcctatcaaggacttcggcggcttcaatttcagccagattctgcccgatcctagcaagcccagcaagcggagcttcatcgaggacctgctgttcaacaaagtgacactggccgacgccggcttcatcaagcagtatggcgattgtctgggcgacattgccgccagggatctgatttgcgcccagaagtttaacggactgacagtgctgcctcctctgctgaccgatgagatgatcgcccagtacacatctgccctgctggccggcacaatcacaagcggctggacatttggagcaggcgccgctctgcagatcccctttgctatgcagatggcctaccggttcaacggcatcggagtgacccagaatgtgctgtacgagaaccagaagctgatcgccaaccagttcaacagcgccatcggcaagatccaggacagcctgagcagcacagcaagcgccctgggaaagctgcagaacgtggtcaaccagaatgcccaggcactgaacaccctggtcaagcagctgtcctccaacttcggcgccatcagctctgtgctgaacgatatcctgagcagactggaccctcctgaggccgaggtgcagatcgacagactgatcacaggcagactgcagagcctccagacatacgtgacccagcagctgatcagagccgccgagattagagcctctgccaatctggccgccaccaagatgtctgagtgtgtgctgggccagagcaagagagtggacttttgcggcaagggctaccacctgatgagcttccctcagtctgcccctcacggcgtggtgtttctgcacgtgacatatgtgcccgctcaagagaagaatttcaccaccgctccagccatctgccacgacggcaaagcccactttcctagagaaggcgtgttcgtgtccaacggcacccattggttcgtgacacagcggaacttctacgagccccagatcatcaccaccgacaacaccttcgtgtctggcaactgcgacgtcgtgatcggcattgtgaacaataccgtgtacgaccctctgcagcccgagctggacagcttcaaagaggaactggacaagtactttaagaaccacacaagccccgacgtggacctgggcgatatcagcggaatcaatgccagcgtcgtgaacatccagaaagagatcgaccggctgaacgaggtggccaagaatctgaacgagagcctgatcgacctgcaagaactggggaagtacgagcagtacatcaagtggccctggtacatctggctgggctttatcgccggactgattgccatcgtgatggtcacaatcatgctgtgttgcatgaccagctgctgtagctgcctgaagggctgttgtagctgtggcagctgctgcaagttcgacgaggacgattctgagcccgtgctgaagggcgtgaaactgcactacacatgatga

SEQ ID NO: 15 - RNA, 4234 nt, synthetic construct
  misc_feature 1..2: note = cap G1G2 = m7G+-5'-ppp-5'-Gm2'-3'-p- [m7 = 7-CH3; m2' = 2'-O-CH3; -ppp- = -PO2H-O-PO2H-O-PO2H)-; -p- = -PO2H-]
  source 1..4234: mol_type = other RNA
ggggaaagctttaatacgactcactataggacagatcgcctggagacgccatccacgctgttttgacctccatagaagacaccgggaccgatccagcctccgcggccgggaacggtgcattggaacgcggattccccgtgccaagagtgacgtaagtaccgcagtcaccgtccttgacacgggatccgccaccatgttcgtgttcctggtgctgctgcctctggtgtccagccagtgtgtgaacctgaggaccagaacacagctgcctccagcctacaccaacagctttaccagaggcgtgtactaccccgacaaggtgttcagatccagcgtgctgcactctacccaggacctgttcctgcctttcttcagcaacgtgacctggttccacgccatccacgtgtccggcaccaatggcaccaagagattcgacaaccccgtgctgcccttcaacgacggggtgtactttgccagcatcgagaagtccaacatcatcagaggctggatcttcggcaccacactggacagcaagacccagagcctgctgatcgtgaacaacgccaccaacgtggtcatcaaagtgtgcgagttccagttctgcaacgaccccttcctggacgtctactaccacaagaacaacaagagctggatggaaagcggcgtgtacagcagcgccaacaactgcaccttcgagtacgtgtcccagcctttcctgatggacctggaaggcaagcagggcaacttcaagaacctgcgcgagttcgtgtttaagaacatcgacggctacttcaagatctacagcaagcacacccctatcaacctcgtgcgggatctgcctcagggcttctctgctctggaacccctggtggatctgcccatcggcatcaacatcacccggtttcagacactgctggccctgcacagaagctacctgacacctggcgatagcagcagcggactgacagctggtgccgccgcttactatgtgggctacctgcagcctagaaccttcctgctgaagtacaacgagaacggcaccatcaccgacgccgtggattgtgctctggaccctctgagcgagacaaagtgcaccctgaagtccttcaccgtggaaaagggcatctaccagaccagcaacttccgggtgcagcccaccgaatccatcgtgcggttccccaatatcaccaatctgtgccccttcggcgaggtgttcaatgccaccagattcgcctctgtgtacgcctggaaccggaagcggatcagcaattgcgtggccgactactccgtgctgtacaactccgccagcttcagcaccttcaagtgctacggcgtgtcccctaccaagctgaacgacctgtgcttcacaaacgtgtacgccgacagcttcgtgatccggggagatgaagtgcggcagattgcccctggacagacaggcaacatcgccgactacaactacaagctgcccgacgacttcaccggctgtgtgattgcctggaacagcaacaacctggactccaaagtcggcggcaactacaattaccggtacaggctgttccggaagtccaatctgaagcccttcgagcgggacatctccaccgagatctatcaggccggcagcaagccttgtaacggcgtggaaggcttcaactgctacttcccactgcagtcctacggctttcagcccacaaatggcgtgggctatcagccctacagagtggtggtgctgagcttcgaactgctgcatgcccctgccacagtgtgcggccctaagaaaagcaccaatctcgtgaagaacaaatgcgtgaacttcaacttcaacggcctgaccggcaccggcgtgctgacagagagcaacaagaagttcctgccattccagcagtttggccgggatatcgccgataccacagacgccgttagagatccccagacactggaaatcctggacatcaccccttgcagcttcggcggagtgtctgtgatcacccctggcaccaacaccagcaatcaggtggcagtgctgtaccagggcgtgaactgtaccgaagtgcccgtggccattcacgccgatcagctgacacctacatggcgggtgtactccaccggcagcaatgtgtttcagaccagagccggctgtctgatcggagccgagcacgtgaacaatagctacgagtgcgacatccccatcggcgctggaatctgcgccagctaccagacacagacaaacagccggcggagagccagaagcgtggccagccagagcatcattgcctacacaatgtctctgggcgccgagaacagcgtggcctactccaacaactctatcgctatccccaccaacttcaccatcagcgtgaccacagagatcctgcctgtgtccatgaccaagaccagcgtggactgcaccatgtacatctgcggcgattccaccgagtgctccaacctgctgctgcagtacggcagcttctgcacccagctgaatagagccctgacagggatcgccgtggaacaggacaagaacacccaagaggtgttcgcccaagtgaagcagatctacaagacccctcctatcaaggacttcggcggcttcaatttcagccagattctgcccgatcctagcaagcccagcaagcggagcttcatcgaggacctgctgttcaacaaagtgacactggccgacgccggcttcatcaagcagtatggcgattgtctgggcgacattgccgccagggatctgatttgcgcccagaagtttaacggactgacagtgctgcctcctctgctgaccgatgagatgatcgcccagtacacatctgccctgctggccggcacaatcacaagcggctggacatttggagcaggcgccgctctgcagatcccctttgctatgcagatggcctaccggttcaacggcatcggagtgacccagaatgtgctgtacgagaaccagaagctgatcgccaaccagttcaacagcgccatcggcaagatccaggacagcctgagcagcacagcaagcgccctgggaaagctgcagaacgtggtcaaccagaatgcccaggcactgaacaccctggtcaagcagctgtcctccaacttcggcgccatcagctctgtgctgaacgatatcctgagcagactggaccctcctgaggccgaggtgcagatcgacagactgatcacaggcagactgcagagcctccagacatacgtgacccagcagctgatcagagccgccgagattagagcctctgccaatctggccgccaccaagatgtctgagtgtgtgctgggccagagcaagagagtggacttttgcggcaagggctaccacctgatgagcttccctcagtctgcccctcacggcgtggtgtttctgcacgtgacatatgtgcccgctcaagagaagaatttcaccaccgctccagccatctgccacgacggcaaagcccactttcctagagaaggcgtgttcgtgtccaacggcacccattggttcgtgacacagcggaacttctacgagccccagatcatcaccaccgacaacaccttcgtgtctggcaactgcgacgtcgtgatcggcattgtgaacaataccgtgtacgaccctctgcagcccgagctggacagcttcaaagaggaactggacaagtactttaagaaccacacaagccccgacgtggacctgggcgatatcagcggaatcaatgccagcgtcgtgaacatccagaaagagatcgaccggctgaacgaggtggccaagaatctgaacgagagcctgatcgacctgcaagaactggggaagtacgagcagtacatcaagtggccctggtacatctggctgggctttatcgccggactgattgccatcgtgatggtcacaatcatgctgtgttgcatgaccagctgctgtagctgcctgaagggctgttgtagctgtggcagctgctgcaagttcgacgaggacgattctgagcccgtgctgaagggcgtgaaactgcactacacatgatgaggtacccgggtggcatccctgtgacccctccccagtgcctctcctggccctggaagttgccactccagtgcccaccagccttgtcctaataaaattaagttgcatcgggcccaaaaaaaaaaaaaaaaaaaaaaaaaaaaaagcatatgactaaaaaaaaaaaaaaaaaaaaaaaaaaaaaaaaaaaaaaaaaaaaaaaaaaaaaaaaaaaaaaaaaaaaaa

SEQ ID NO: 16 - DNA, 38 bp, synthetic construct
  misc_feature 1..38: note = 5'UTR
  source 1..38: mol_type = other DNA
agagactgcgagaaggaggtcccccacggcccttcagg

SEQ ID NO: 17 - DNA, 27 bp, synthetic construct
  misc_feature 1..27: note = 5'UTR
  source 1..27: mol_type = other DNA
acacaagaagggtaggagagaaaagcc

SEQ ID NO: 18 - DNA, 73 bp, synthetic construct
  misc_feature 1..73: note = 5'UTR
  source 1..73: mol_type = other DNA
agtatattagtgctaatttccctccgtttgtcctagcttttctcttctgtcaaccccacacgcctttggcaca

SEQ ID NO: 19 - DNA, 90 bp, synthetic construct
  misc_feature 1..90: note = 5'UTR
  source 1..90: mol_type = other DNA
ctccccagcctgataaaggtcctgcgggcaggacaggacctcccaaccaagccctccagcaaggattcagagtgcccctccggcctcgcc

SEQ ID NO: 20 - DNA, 63 bp, synthetic construct
  misc_feature 1..63: note = 5'UTR
  source 1..63: mol_type = other DNA
ctttttcgcaacgggtttgccgccagaacacaggtgtcgtgaaaactacccctaaaagccaaa

SEQ ID NO: 21 - DNA, 84 bp, synthetic construct
  misc_feature 1..84: note = 5'UTR
  source 1..84: mol_type = other DNA
cgcctccctcgctccacgcgcgcccggactcggcggccaggcttgcgcgcggttcccctcccggtgggcggattcctgggcaag

SEQ ID NO: 22 - DNA, 34 bp, synthetic construct
  misc_feature 1..34: note = 5'UTR
  source 1..34: mol_type = other DNA
agttccccaaagataacacagctttgcacagtgg

SEQ ID NO: 23 - DNA, 67 bp, synthetic construct
  misc_feature 1..67: note = 5'UTR
  source 1..67: mol_type = other DNA
cggggcggggccgcgtgacgtgccgggaagccggagtctagagctccgggcgcggggaggcgcggcc

SEQ ID NO: 24 - DNA, 65 bp, synthetic construct
  misc_feature 1..65: note = 5'UTR
  source 1..65: mol_type = other DNA
gtggaagcggacctgaggagtcgcaattgtgaacaggttcggtgctgcggctggggctcagcgat

SEQ ID NO: 25 - DNA, 98 bp, synthetic construct
  misc_feature 1..98: note = 5'UTR
  source 1..98: mol_type = other DNA
gggagtcggagaaaaagctgacctaatgaaactgtggcaacgtcagcgcttgaggcttgaagagggagacaagctaaaagaggatatccagttgtttc

SEQ ID NO: 26 - DNA, 95 bp, synthetic construct
  misc_feature 1..95: note = 5'UTR
  source 1..95: mol_type = other DNA
cagaggaggagctcgctgccgggggacgctgggctgagcggccggcggcgcggccccggcggcggcggcagcggggtccgggtccggagcgccac

SEQ ID NO: 27 - DNA, 91 bp, synthetic construct
  misc_feature 1..91: note = 5'UTR
  source 1..91: mol_type = other DNA
gcgggcggcgggcggagctggtcccgttgtgctgcggccccgcgcggcctgcagtcccgggctcgcgccccgcgccgcccgcccgcccgcc

SEQ ID NO: 28 - DNA, 64 bp, synthetic construct
  misc_feature 1..64: note = 5'UTR
  source 1..64: mol_type = other DNA
acggcttacccgggctccgacagcggctgcaggagcccaagttgcggccgctggagcccgagcc

SEQ ID NO: 29 - DNA, 84 bp, synthetic construct
  misc_feature 1..84: note = 5'UTR
  source 1..84: mol_type = other DNA
accgccgagacagcgtccgccccgcgagcacagagcctcgcctttgccgatccgccgcccgtccacacccgccgccagctcacc

SEQ ID NO: 30 - DNA, 245 bp, synthetic construct
  misc_feature 1..245: note = 5'UTR
  source 1..245: mol_type = other DNA
cggctcctctcagcggcggtggcccaggtagaggggtccgcgctggcggcggcggcggcgctgttccccgcgcggtccgcggagcggggtccgggctgcgcgacgtggggcggcggcggcactgcggccccggcccaagcccgaccccgggtcccctcctcggccgccccccgcccggccgcccgccctcgggcctccccccgaaccctcggtcccctcccccgctggcggggaacggacagaag

SEQ ID NO: 31 - DNA, 112 bp, synthetic construct
  misc_feature 1..112: note = 5'UTR
  source 1..112: mol_type = other DNA
acagagtaaacttttgctgggctccaagtgaccgcccatagtttattataaaggtgactgcaccctgcagccaccagcactgcctggctccacgtgcctcctggtctcagtg

SEQ ID NO: 32 - DNA, 102 bp, synthetic construct
  misc_feature 1..102: note = 5'UTR
  source 1..102: mol_type = other DNA
aaattgagcccgcagcctcccgcttcgctctctgctcctcctgttcgacagtcagccgcatcttcttttgcgtcgccagccgagccacatcgctcagacacc

SEQ ID NO: 33 - DNA, 127 bp, synthetic construct
  misc_feature 1..127: note = 5'UTR
  source 1..127: mol_type = other DNA
gttactagaagggctccaggatggaggccgacctgacttctccgcctcggtgggctgggtcggcggctggagcattacccctactgcgggtcccgctgctggcagcgctggaaactgggtggacggc

SEQ ID NO: 34 - DNA, 150 bp, synthetic construct
  misc_feature 1..150: note = 5'UTR
  source 1..150: mol_type = other DNA
tgactgcagcagcagcggcagcgcctcggttcctgagcccaccgcaggctgaaggcattgcgcgtagtccatgcccgtagaggaagtgtgcagatgggattaacgtccacatggagatatggaagaggaccggggattggaaccgtaacc

SEQ ID NO: 35 - DNA, 162 bp, synthetic construct
  misc_feature 1..162: note = 5'UTR
  source 1..162: mol_type = other DNA
tggtgacgtcacggcgctcgtcggcgccgcctgtggcgtcacaggccgggaacgcagggctttctaggggtccgtcgctcttgaagccgccggcggcgggcgcgtgcgcggcccgatgaagaaggaggtttccaagccgtctccgcccaagttgatcggtgg

SEQ ID NO: 36 - DNA, 148 bp, synthetic construct
  misc_feature 1..148: note = 5'UTR
  source 1..148: mol_type = other DNA
ggtgagtggcccctgctggaccgtgaatcccgggcgggcgtgcgggcggcagcgtacgaggccttctactcgcccgggtgtccggtgcctcgcttctccctgggaccctgtcgtcaacatcgaggcctgccagtgagcttctaccatc

SEQ ID NO: 37 - DNA, 126 bp, synthetic construct
  misc_feature 1..126: note = 5'UTR
  source 1..126: mol_type = other DNA
gtagtggtgccgacttcctgttgtttgaggccgggttgggggtgtgcgattgtgtgggacggtctggggcagcccagcagcggctgaccctctgcctgcggggaagggagtcgccaggcggccgtc

SEQ ID NO: 38 - DNA, 114 bp, synthetic construct
  misc_feature 1..114: note = 5'UTR
  source 1..114: mol_type = other DNA
gaactcgggttgcgcacttcccggcgctgggaacgcggagcggacgcagtctggccgccattgcgctgcggggaaagcggcctcttgtgtgagggcctgtgggattctccggat

SEQ ID NO: 39 - DNA, 194 bp, synthetic construct
  misc_feature 1..194: note = 5'UTR
  source 1..194: mol_type = other DNA
ggtattttcgggactttcctaagctgctctaactttcctgccccttccccggccaagcccaactccggatctcgctctccaccggatctcacccgccacacccggacaggcggctggaggaggcgggcgtctaaaattctgggaagcagaacctggccggagccactagacagagccgggcctagcccagagac

SEQ ID NO: 40 - DNA, 193 bp, synthetic construct
  misc_feature 1..193: note = 5'UTR
  source 1..193: mol_type = other DNA
agtgcgcctgcgcgcttgtggagctggtggcggcgctccgcaggggctcggctgttttccgcgcggcaggcgcggccatggcgcagctgggaaagctgctcaaggagcagaagtacgaccggcagctgaggcgattcctccatacatttgacagctgtctgaacccttatggagcatacagtggagtggaaag

SEQ ID NO: 41 - DNA, 127 bp, synthetic construct
  misc_feature 1..127: note = 5'UTR
  source 1..127: mol_type = other DNA
ttaggtggcgccggtcccctcgaacaggtcgctcaacaactcccgcccagcagccgcccttactgcgcgcgcgcagacttcggcgtctacttccggtgtggcccaggcggggtccgcagaaccagct

SEQ ID NO: 42 - DNA, 134 bp, synthetic construct
  misc_feature 1..134: note = 5'UTR
  source 1..134: mol_type = other DNA
cctgggcaagccctgcgtcaggttgcagtttcacttttagctctgggcacctccagctcctgctcgccggacggctcccagggagagcagacgcgccagacgcgccaccctcggggcgccgacggtcacggagc

SEQ ID NO: 43 - DNA, 186 bp, synthetic construct
  misc_feature 1..186: note = 5'UTR
  source 1..186: mol_type = other DNA
ttctttctcctccactgcaaagttaaatgcgagaaggtagaaacccagaggccatgctggcgctgagagatgagccccactcaccagattcaagatcccaagtgctgcagactttggcaaagcctataaattcagagcagcccggagaggagaaaggaaagtggatgtgggttcaggccgcatgaa

SEQ ID NO: 44 - DNA, 232 bp, synthetic construct
  misc_feature 1..232: note = 5'UTR
  source 1..232: mol_type = other DNA
acggtaaagccatgtttccaaggaggtctgtacaaaaagccagacttctgctggcagttactgagagagataggctttccatccatggcagccatttacttttgctctgggagacgtttgtaatagaaaaggcacaactggggtatttattcattccccccgttcctctagtgtttggtggcgttgccgttgcaagtgcgcagggctaaaatggactggttatcttaggatc

SEQ ID NO: 45 - DNA, 120 bp, synthetic construct
  misc_feature 1..120: note = 5'UTR
  source 1..120: mol_type = other DNA
gcttcccgtccgctgtcctctgctgccagtcccctgccccgggcaaagcccatctggtccgccgagcaggccggagctattgggagtggcgcatcctcccaccccagccggatctgggcc

SEQ ID NO: 46 - DNA, 120 bp, synthetic construct
  misc_feature 1..120: note = 5'UTR
  source 1..120: mol_type = other DNA
ctggggacgggggccgagtagcgccttccccgggccccgtgaaccggctgcgggtcgcccttggggggcagcggccgcagccccccacctgggccctcggtccgccctcccggcgcgtcc

SEQ ID NO: 47 - DNA, 55 bp, synthetic construct
  misc_feature 1..55: note = 3'UTR
  source 1..55: mol_type = other DNA
ggcgcccgccgccgccccccttcccggtgctcagaataaacgtttccaaagtggg

SEQ ID NO: 48 - DNA, 93 bp, synthetic construct
  misc_feature 1..93: note = 3'UTR
  source 1..93: mol_type = other DNA
actattgtatatatatcagttactgttatggaccccacgtcactattgtatactctatattatactctatgttatactctgtaatcctactca

SEQ ID NO: 49 - DNA, 74 bp, synthetic construct
  misc_feature 1..74: note = 3'UTR
  source 1..74: mol_type = other DNA
tcttcacccagtctgtctcttagaatttatttcccactgacacaaacaagccattttgtctgcttgtataaccc

SEQ ID NO: 50 - DNA, 79 bp, synthetic construct
  misc_feature 1..79: note = 3'UTR
  source 1..79: mol_type = other DNA
ttattttaaagttaagacattttaatcttgacacagtagatcttactttcaaagttataaacttgaagtgattgtagtt

SEQ ID NO: 51 - DNA, 79 bp, synthetic construct; identical to SEQ ID NO: 50
  misc_feature 1..79: note = 3'UTR
  source 1..79: mol_type = other DNA

SEQ ID NO: 52 - DNA, 81 bp, synthetic construct
  misc_feature 1..81: note = 3'UTR
  source 1..81: mol_type = other DNA
atgcattatggtcaaatcttttcatgtatatggatgtgactattttaacaaataaaagaagtgaaaagttatttaccttgt

SEQ ID NO: 53 - DNA, 198 bp, synthetic construct
  misc_feature 1..198: note = 3'UTR
  source 1..198: mol_type = other DNA
ccaggttctacagggaggctgcacccactccatgttacttctgcttcgctttcccctaccccccccccataaagacaaaccaatcaaccacgacaaaggaagttgacctgaacatgtaaccatgccctaccctgttaccttgctagctgcaaaataaacttgttgctgacctgctgtgctcgcagtagattccaagtt

SEQ ID NO: 54 - DNA, 132 bp, synthetic construct
  misc_feature 1..132: note = 3'UTR
  source 1..132: mol_type = other DNA
gctcgctttcttgctgtccaatttctattaaaggttcctttgttccctaagtccaactactaaactgggggatattatgaagggccttgagcatctggattctgcctaataaaaaacatttattttcattgc

SEQ ID NO: 55 - DNA, 386 bp, synthetic construct
  misc_feature 1..386: note = 3'UTR
  source 1..386: mol_type = other DNA
aatctcagaggtagggctgccaccaaggtgaagatgggaacgcagatgatccatgagtttgccctggtttcactggcccaagtggtttgtgctaaccacgtctgtcttcacagctctgtgttgccatgtgtgctgaacaaaaaataaaaattattattgattttatatttcaaaaactccattctttcctaaatattttcaacaaaggatttctttatgcattctgcctaaatacctatgcaactgagcccttccttctcagctcaagattcgtctggtctttccctacagctttgtgtgtgccatggccacatctcctgggtacagttcaaggagacatcttttctaaaagggtctgcgtgatcattaaaatataatcaaatgta

SEQ ID NO: 56 - DNA, 416 bp, synthetic construct
  misc_feature 1..416: note = 3'UTR
  source 1..416: mol_type = other DNA
tgaggcgtgcgccgccaatatgcactgtacattccacaagcattgccttcttattttacttcttttagctgtttaactttgtaagatgcaaagaggttggatcaagtttaaatgactgtgctgcccctttcacatcaaagaactactgacaacgaaggccgcgcctgcctttcccatctgtctatctatctggctggcagggaaggaaagaacttgcatgttggtgaaggaagaagtggggtggaagaagtggggtgggacgacagtgaaatctagagtaaaaccaagctggcccaaggtgtcctgcaggctgtaatgcagtttaatcagagtgccatttttttttttgttcaaatgattttaattattggaatgcacaatttttttaatatgcaaataaaaagtttaaaaactta

SEQ ID NO: 57 - DNA, 156 bp, synthetic construct
  misc_feature 1..156: note = 3'UTR
  source 1..156: mol_type = other DNA
tcctacaaccacatgcagttgtgggaccgcagtttggtcctggggaccattcatacccacacacccagcttgtgcctgtggttaacatctcagaaaactctggtaaatgatcactccaggatattgacaagaatacacgttactgatcttactcac

SEQ ID NO: 58 - DNA, 322 bp, synthetic construct
  misc_feature 1..322: note = 3'UTR
  source 1..322: mol_type = other DNA
aaattgcacacactcagtgcagcaatatattaccagcaagaataaaaaagaaatccatatcttaaagaaacagctttcaagtgcctttctgcagtttttcaggagcgcaagatagatttggaataggaataagctctagttcttaacaaccgacactcctacaagatttagaaaaaagtttacaacataatctagtttacagaaaaatcttgtgctagaatactttttaaaaggtattttgaataccattaaaactgcttttttttttccagcaagtatccaaccaacttggttctgcttcaataaatctttggaaaaactc

SEQ ID NO: 59 - DNA, 189 bp, synthetic construct
  misc_feature 1..189: note = 3'UTR
  source 1..189: mol_type = other DNA
ttaccagcgtttccagaagagcccctgccccgttcctgctgcggcctggccgttcttggggaatctgaccacggcgtgcaaactgggactgcctttccctctcctcagcccgtcctcctccaacccgcgctcctttgccctgccgggcaacaggatggcaggccacctgactctcacctctgtgccccc

SEQ ID NO: 60 - DNA, 348 bp, synthetic construct
  misc_feature 1..348: note = 3'UTR
  source 1..348: mol_type = other DNA
gggacttctcctccagtggacctgaaggacgagggatgggatttcatgtaaccaagagtattccatttttactaaagcagtgttttcacctcatatgctatgttagaagtccaggcagagacaataaaacattcctgtgaaaggcacttttcattccactttaacttgattttttaaattcccttattgtcccttccaaaaaaaagagaatcaaaattttacaaagaatcaaaggattctagaaagtatctgggcagaacgctaggagagatccaaatttccattgtcttgcaagcaaagcacgtattaaatatgatctgcagccattaaaaagacacattctgtaaa

SEQ ID NO: 61 - DNA, 273 bp, synthetic construct
  misc_feature 1..273: note = 3'UTR
  source 1..273: mol_type = other DNA
gcccaggcgccaccactgatgccacccaggacctcggaccttggagcctgcggggtgcctcggcccctccagccccgggccggacctcctgctggctctcgcccaccaaccaagtgttacaagccccagaatgctgcccggcctgccctgctgggcggactgtctgtgtgtctgtctctctggcgttccacctccaagcctataccagctgtgtacagcgccatctctctgccttctgttgcccctcactcaccaaacacgtgtatttatagc

SEQ ID NO: 62 - DNA, 110 bp, synthetic construct
  misc_feature 1..110: note = 3'UTR
  source 1..110: mol_type = other DNA
gctggagcctcggtggccatgcttcttgccccttgggcctccccccagcccctcctccccttcctgcacccgtacccccgtggtctttgaataaagtctgagtgggcggc

SEQ ID NO: 63 - DNA, 172 bp, synthetic construct
  misc_feature 1..172: note = 3'UTR
  source 1..172: mol_type = other DNA
ccgtttccctgcctcctgcttcagcctcccgaggccgaagcctcagcccctccagacaggccgctgacattcagcagtttggcctctttccctctgtctgtgcttgtgttgttgacctcctgatggcttgtcatcctgaataaaatataataataaattttgtataaatagg

SEQ ID NO: 64 - DNA, 299 bp, synthetic construct
  misc_feature 1..299: note = 3'UTR
  source 1..299: mol_type = other DNA
cagccttctgtcttaaaggttttataatgctgactgaatatctgttatgcatttttaaagtattaaactaacattaggatttgctaactagctttcatcaaaaatgggagcatggctataagacaactatattttattatatgttttctgaagtaacattgtatcatagattaacattttaaattaccataatcatgctatgtaaatataagactactggctttgtgagggaatgtttgtgcaaaattttttcctctaatgtataatagtgttaaattgattaaaaatcttccagaatt

SEQ ID NO: 65 - DNA, 239 bp, synthetic construct
  misc_feature 1..239: note = 3'UTR
  source 1..239: mol_type = other DNA
catctggtccaacatgaaaacaattcttattgactcatacaccaggtcacgctttcatgagttctgtcatttcaaagactctcacccctgctataactatgaccatgctgataaactgatttatctatttaaatatttatttaactattcataagatttaaattatttttgttcatataacgtcatgtgcacctttacactgtggttagtgtaataaaacatgttccttatatttactc

SEQ ID NO: 66 - DNA, 336 bp, synthetic construct
  misc_feature 1..336: note = 3'UTR
  source 1..336: mol_type = other DNA
atatgtgaacaaatccaggcctctcaaggaaaagacttcaaccaggcttccttgtacccacaggtgaaaaatgtgagcataatacttctaatattattgataagtaaggtaaccacaattagtcagcaacagagtacaacagggtttctatttacccaccaactactatacctttcatgacgttgaatgggacatagaactgtcctacatttatgtcaaagtatatatttgaatcgcttatattttctttttcactctttatattgagtacattccagaaatttgtagtaggcaaggtgctataaaaatgcactaaaaataaatctgttctcaatg

SEQ ID NO: 67 - DNA, 125 bp, synthetic construct
  misc_feature 1..125: note = 3'UTR
  source 1..125: mol_type = other DNA
tcgcccacaagccttactcacctctctctaagtttagaagcgctcatctggcttttcgcttgcttctgcagcaactcccacgactgttgtacaagctcaggaggcgaataaatgttcaaactgta

SEQ ID NO: 68 - DNA, 110 bp, synthetic construct
  misc_feature 1..110: note = polyA
  source 1..110: mol_type = other DNA
aaaaaaaaaaaaaaaaaaaaaaaaaaaaaagcatatgtcaaaaaaaaaaaaaaaaaaaaaaaaaaaaaaaaaaaaaaaaaaaaaaaaaaaaaaaaaaaaaaaaaaaaaaa

SEQ ID NO: 69 - DNA, 110 bp, synthetic construct
  misc_feature 1..110: note = polyA
  source 1..110: mol_type = other DNA
aaaaaaaaaaaaaaaaaaaaaaaaaaaaaagcatatcagtaaaaaaaaaaaaaaaaaaaaaaaaaaaaaaaaaaaaaaaaaaaaaaaaaaaaaaaaaaaaaaaaaaaaaa

SEQ ID NO: 70 - DNA, 110 bp, synthetic construct
  misc_feature 1..110: note = polyA
  source 1..110: mol_type = other DNA
aaaaaaaaaaaaaaaaaaaaaaaaaaaaaacgatatgactaaaaaaaaaaaaaaaaaaaaaaaaaaaaaaaaaaaaaaaaaaaaaaaaaaaaaaaaaaaaaaaaaaaaaa

SEQ ID NO: 71 - DNA, 110 bp, synthetic construct
  misc_feature 1..110: note = polyA
  source 1..110: mol_type = other DNA
aaaaaaaaaaaaaaaaaaaaaaaaaaaaaacgatgatactaaaaaaaaaaaaaaaaaaaaaaaaaaaaaaaaaaaaaaaaaaaaaaaaaaaaaaaaaaaaaaaaaaaaaa

SEQ ID NO: 72 - DNA, 108 bp, synthetic construct
  misc_feature 1..108: note = polyA
  source 1..108: mol_type = other DNA
aaaaaaaaaaaaaaaaaaaaaaaaaaaaaacggttgggaaaaaaaaaaaaaaaaaaaaaaaaaaaaaaaaaaaaaaaaaaaaaaaaaaaaaaaaaaaaaaaaaaaaaa

SEQ ID NO: 73 - DNA, 113 bp, synthetic construct
  misc_feature 1..113: note = polyA
  source 1..113: mol_type = other DNA
aaaaaaaaaaaaaaaaaaaaaaaaaaaaaaaatttcggttgggaaaaaaaaaaaaaaaaaaaaaaaaaaaaaaaaaaaaaaaaaaaaaaaaaaaaaaaaaaaaaaaaaaaaaa

SEQ ID NO: 74 - DNA, 110 bp, synthetic construct
  misc_feature 1..110: note = polyA
  source 1..110: mol_type = other DNA
aaaaaaaaaaaaaaaaaaaaaaaaaaaaaacagcgtatataaaaaaaaaaaaaaaaaaaaaaaaaaaaaaaaaaaaaaaaaaaaaaaaaaaaaaaaaaaaaaaaaaaaaa

SEQ ID NO: 75 - DNA, 110 bp, synthetic construct
  misc_feature 1..110: note = polyA
  source 1..110: mol_type = other DNA
aaaaaaaaaaaaaaaaaaaaaaaaaaaaaagatatgcactaaaaaaaaaaaaaaaaaaaaaaaaaaaaaaaaaaaaaaaaaaaaaaaaaaaaaaaaaaaaaaaaaaaaaa

SEQ ID NO: 76 - DNA, 120 bp, synthetic construct
  misc_feature 1..120: note = polyA
  source 1..120: mol_type = other DNA
aaaaaaaaaaaaaaaaaaaaaaaaaaaaaacatgtacgataaaaaaaaaaaaaaaaaaaaaaaaaaaaaagatatgcactaaaaaaaaaaaaaaaaaaaaaaaaaaaaaaaaaaaaaaaa